European Patent Specification EP 4 048 315 B1, published March 12, 2025. Title: THIENOAZEPINE IMMUNOCONJUGATES, AND USES THEREOF. Applicant: BOLT BIOTHERAPEUTICS, INC. The sequence listing filed with the application follows.

SEQUENCE LISTING (607 sequences)

SEQ ID NO: 1 - protein, 5 aa, Artificial Sequence
  source: /note="Description of Artificial Sequence: Synthetic peptide"
SYAIS

SEQ ID NO: 2 - protein, 5 aa, Artificial Sequence
  source: /note="Description of Artificial Sequence: Synthetic peptide"
SYYMH

SEQ ID NO: 3 - protein, 5 aa, Artificial Sequence
  source: /note="Description of Artificial Sequence: Synthetic peptide"
RHLLH

SEQ ID NO: 4 - protein, 5 aa, Artificial Sequence
  source: /note="Description of Artificial Sequence: Synthetic peptide"
SHHMH

SEQ ID NO: 5 - protein, 4 aa, Artificial Sequence
  source: /note="Description of Artificial Sequence: Synthetic peptide"
RFMH

SEQ ID NO: 6 - protein, 5 aa, Artificial Sequence
  source: /note="Description of Artificial Sequence: Synthetic peptide"
SYYIH

SEQ ID NO: 7 - protein, 5 aa, Artificial Sequence
  source: /note="Description of Artificial Sequence: Synthetic peptide"
NYYIH

SEQ ID NO: 8 - protein, 5 aa, Artificial Sequence
  source: /note="Description of Artificial Sequence: Synthetic peptide"
HYYMH

SEQ ID NO: 9 - protein, 5 aa, Artificial Sequence
  source: /note="Description of Artificial Sequence: Synthetic peptide"
GYYMH

SEQ ID NO: 10 - protein, 5 aa, Artificial Sequence
  source: /note="Description of Artificial Sequence: Synthetic peptide"
NYMYH

SEQ ID NO: 11 - protein, 5 aa, Artificial Sequence
  source: /note="Description of Artificial Sequence: Synthetic peptide"
TYYVH

SEQ ID NO: 12 - protein, 5 aa, Artificial Sequence
  source: /note="Description of Artificial Sequence: Synthetic peptide"
SYALS

SEQ ID NO: 13 - protein, 5 aa, Artificial Sequence
  source: /note="Description of Artificial Sequence: Synthetic peptide"
RHYVH

SEQ ID NO: 14 - protein, 5 aa, Artificial Sequence
  source: /note="Description of Artificial Sequence: Synthetic peptide"
SHYMH

SEQ ID NO: 15 - protein, 5 aa, Artificial Sequence
  source: /note="Description of Artificial Sequence: Synthetic peptide"
DYYMH

SEQ ID NO: 16 - protein, 5 aa, Artificial Sequence
  source: /note="Description of Artificial Sequence: Synthetic peptide"
GYTLH

SEQ ID NO: 17 - protein, 5 aa, Artificial Sequence
  source: /note="Description of Artificial Sequence: Synthetic peptide"
NHYMH

SEQ ID NO: 18 - protein, 5 aa, Artificial Sequence
  source: /note="Description of Artificial Sequence: Synthetic peptide"
NSYMH

SEQ ID NO: 19 - protein, 5 aa, Artificial Sequence
  source: /note="Description of Artificial Sequence: Synthetic peptide"
TYYMH

SEQ ID NO: 20 - protein, 5 aa, Artificial Sequence
  source: /note="Description of Artificial Sequence: Synthetic peptide"
RHFIH

SEQ ID NO: 21 - protein, 5 aa, Artificial Sequence
  source: /note="Description of Artificial Sequence: Synthetic peptide"
TFGIS

SEQ ID NO: 22 - protein, 5 aa, Artificial Sequence
  source: /note="Description of Artificial Sequence: Synthetic peptide"
SYGIN

SEQ ID NO: 23 - protein, 5 aa, Artificial Sequence
  source: /note="Description of Artificial Sequence: Synthetic peptide"
NHYVH

SEQ ID NO: 24 - protein, 17 aa, Artificial Sequence
  source: /note="Description of Artificial Sequence: Synthetic peptide"
VINPSAGSTDYAQKFQG

SEQ ID NO: 25 - protein, 17 aa, Artificial Sequence
  source: /note="Description of Artificial Sequence: Synthetic peptide"
WMNPNSDIAGYAQKFQG

SEQ ID NO: 26 - protein, 17 aa, Artificial Sequence
  source: /note="Description of Artificial Sequence: Synthetic peptide"
WISPQHGVRNYAQKFQG

SEQ ID NO: 27 - protein, 17 aa, Artificial Sequence
  source: /note="Description of Artificial Sequence: Synthetic peptide"
WVSPSHGLTGYAQKFQG

SEQ ID NO: 28 - protein, 17 aa, Artificial Sequence
  source: /note="Description of Artificial Sequence: Synthetic peptide"
WMSLNSGLTGYAQKFQG

SEQ ID NO: 29 - protein, 17 aa, Artificial Sequence
  source: /note="Description of Artificial Sequence: Synthetic peptide"
WMKPSSGTTGYAQKFQG

SEQ ID NO: 30 - protein, 17 aa, Artificial Sequence
  source: /note="Description of Artificial Sequence: Synthetic peptide"
WMNPNGDVAGYAQKFQG

SEQ ID NO: 31 - protein, 17 aa, Artificial Sequence
  source: /note="Description of Artificial Sequence: Synthetic peptide"
GIDPNSGGTNYAQKFQG

SEQ ID NO: 32 - protein, 17 aa, Artificial Sequence
  source: /note="Description of Artificial Sequence: Synthetic peptide"
WMNPDSGSTGYAQKFQG

SEQ ID NO: 33 - protein, 17 aa, Artificial Sequence
  source: /note="Description of Artificial Sequence: Synthetic peptide"
WMSLNSGLTGYAQKFQG

SEQ ID NO: 34 - protein, 17 aa, Artificial Sequence
  source: /note="Description of Artificial Sequence: Synthetic peptide"
WMNPNGDVAGYADSFQG

SEQ ID NO: 35 - protein, 17 aa, Artificial Sequence
  source: /note="Description of Artificial Sequence: Synthetic peptide"
WISTYHGSTNYAQKFQG

SEQ ID NO: 36 - protein, 17 aa, Artificial Sequence
  source: /note="Description of Artificial Sequence: Synthetic peptide"
WMNPNTVYTGSAQKFQG

SEQ ID NO: 37 - protein, 17 aa, Artificial Sequence
  source: /note="Description of Artificial Sequence: Synthetic peptide"
RIIPAVGSVTYAQKFQG

SEQ ID NO: 38 - protein, 17 aa, Artificial Sequence
  source: /note="Description of Artificial Sequence: Synthetic peptide"
GIIPIFGTANYAQKFQG

SEQ ID NO: 39 - protein, 17 aa, Artificial Sequence
  source: /note="Description of Artificial Sequence: Synthetic peptide"
WMSPSSGITGYAQKFQG

SEQ ID NO: 40 - protein, 17 aa, Artificial Sequence
  source: /note="Description of Artificial Sequence: Synthetic peptide"
WMTPSTGNAGYAQKFQG

SEQ ID NO: 41 - protein, 17 aa, Artificial Sequence
  source: /note="Description of Artificial Sequence: Synthetic peptide"
WMNPNSGNTGYAQKFQG

SEQ ID NO: 42 - protein, 17 aa, Artificial Sequence
  source: /note="Description of Artificial Sequence: Synthetic peptide"
WMHPNSGHTGYAQKFQG

SEQ ID NO: 43 - protein, 17 aa, Artificial Sequence
  source: /note="Description of Artificial Sequence: Synthetic peptide"
WMNPNSGHTGNAQKFQG

SEQ ID NO: 44 - protein, 17 aa, Artificial Sequence
  source: /note="Description of Artificial Sequence: Synthetic peptide"
WIDPNSGVTSSAQKFQG

SEQ ID NO: 45 - protein, 17 aa, Artificial Sequence
  source: /note="Description of Artificial Sequence: Synthetic peptide"
WISPNSGVTDFTQKFQG

SEQ ID NO: 46 - protein, 17 aa, Artificial Sequence
  source: /note="Description of Artificial Sequence: Synthetic peptide"
WMNPNSGHTGYAQRFQG

SEQ ID NO: 47 - protein, 17 aa, Artificial Sequence
  source: /note="Description of Artificial Sequence: Synthetic peptide"
WMSPNGGNTGYAQKFQG

SEQ ID NO: 48 - protein, 17 aa, Artificial Sequence
  source: /note="Description of Artificial Sequence: Synthetic peptide"
WMDPSSGYTGSAHKFQG

SEQ ID NO: 49 - protein, 17 aa, Artificial Sequence
  source: /note="Description of Artificial Sequence: Synthetic peptide"
WMNPHSADTGYAEKFQG

SEQ ID NO: 50 - protein, 17 aa, Artificial Sequence
  source: /note="Description of Artificial Sequence: Synthetic peptide"
WLTPSTGHAGYAQKFQG

SEQ ID NO: 51 - protein, 17 aa, Artificial Sequence
  source: /note="Description of Artificial Sequence: Synthetic peptide"
WMNPNSGHTGYAQKFQG

SEQ ID NO: 52 - protein, 17 aa, Artificial Sequence
  source: /note="Description of Artificial Sequence: Synthetic peptide"
WISPQHGVRNYAHKFQG

SEQ ID NO: 53 - protein, 17 aa, Artificial Sequence
  source: /note="Description of Artificial Sequence: Synthetic peptide"
MINPSGGSTSYAQKFQG

SEQ ID NO: 54 - protein, 17 aa, Artificial Sequence
  source: /note="Description of Artificial Sequence: Synthetic peptide"
WISPRSGVTSYAQKFQG

SEQ ID NO: 55 - protein, 17 aa, Artificial Sequence
  source: /note="Description of Artificial Sequence: Synthetic peptide"
WMDPNSGNTGYAQKFQG

SEQ ID NO: 56 - protein, 17 aa, Artificial Sequence
  source: /note="Description of Artificial Sequence: Synthetic peptide"
WMNPTGGITGYAQKFQG

SEQ ID NO: 57 - protein, 17 aa, Artificial Sequence
  source: /note="Description of Artificial Sequence: Synthetic peptide"
WVSPIHGLTGYAPRFQG

SEQ ID NO: 58 - protein, 18 aa, Artificial Sequence
  source: /note="Description of Artificial Sequence: Synthetic peptide"
DLYPYVVVVAAGSYGMDV

SEQ ID NO: 59 - protein, 12 aa, Artificial Sequence
  source: /note="Description of Artificial Sequence: Synthetic peptide"
PSIVGAYDAFDI

SEQ ID NO: 60 - protein, 9 aa, Artificial Sequence
  source: /note="Description of Artificial Sequence: Synthetic peptide"
ESVEGYFDL

SEQ ID NO: 61 - protein, 11 aa, Artificial Sequence
  source: /note="Description of Artificial Sequence: Synthetic peptide"
DNWNVHDAFDI

SEQ ID NO: 62 - protein, 9 aa, Artificial Sequence
  source: /note="Description of Artificial Sequence: Synthetic peptide"
GTYNDAFDI

SEQ ID NO: 63 - protein, 11 aa, Artificial Sequence
  source: /note="Description of Artificial Sequence: Synthetic peptide"
EQWLVNDAFDI

SEQ ID NO: 64 - protein, 13 aa, Artificial Sequence
  source: /note="Description of Artificial Sequence: Synthetic peptide"
DSSGWMRNDAFDI

SEQ ID NO: 65 - protein, 14 aa, Artificial Sequence
  source: /note="Description of Artificial Sequence: Synthetic peptide"
SMFPTIFGDNAFDI

SEQ ID NO: 66 - protein, 14 aa, Artificial Sequence
  source: /note="Description of Artificial Sequence: Synthetic peptide"
ALFPYPFYYYYMDV

SEQ ID NO: 67 - protein, 7 aa, Artificial Sequence
  source: /note="Description of Artificial Sequence: Synthetic peptide"
DRGWFDP

SEQ ID NO: 68 - protein, 10 aa, Artificial Sequence
  source: /note="Description of Artificial Sequence: Synthetic peptide"
DARGYSGYDL

SEQ ID NO: 69 - protein, 9 aa, Artificial Sequence
  source: /note="Description of Artificial Sequence: Synthetic peptide"
EGRHGEYLY

SEQ ID NO: 70 - protein, 11 aa, Artificial Sequence
  source: /note="Description of Artificial Sequence: Synthetic peptide"
EGWGSSGYFDY

SEQ ID NO: 71 - protein, 15 aa, Artificial Sequence
  source: /note="Description of Artificial Sequence: Synthetic peptide"
HLFPTVFDDYYGMDV

SEQ ID NO: 72 - protein, 10 aa, Artificial Sequence
  source: /note="Description of Artificial Sequence: Synthetic peptide"
GGYSYGSFQH

SEQ ID NO: 73 - protein, 10 aa, Artificial Sequence
  source: /note="Description of Artificial Sequence: Synthetic peptide"
VRWSSDAFDI

SEQ ID NO: 74 - protein, 9 aa, Artificial Sequence
  source: /note="Description of Artificial Sequence: Synthetic peptide"
EEWLGHFQH

SEQ ID NO: 75 - protein, 9 aa, Artificial Sequence
  source: /note="Description of Artificial Sequence: Synthetic peptide"
ERFLGGMDV

SEQ ID NO: 76 - protein, 9 aa, Artificial Sequence
  source: /note="Description of Artificial Sequence: Synthetic peptide"
GNWVDAFDI

SEQ ID NO: 77 - protein, 11 aa, Artificial Sequence
  source: /note="Description of Artificial Sequence: Synthetic peptide"
ESEVMMAYFQH

SEQ ID NO: 78 - protein, 9 aa, Artificial Sequence
  source: /note="Description of Artificial Sequence: Synthetic peptide"
ESWSGEFDY

SEQ ID NO: 79 - protein, 9 aa, Artificial Sequence
  source: /note="Description of Artificial Sequence: Synthetic peptide"
EAVAGPMDV

SEQ ID NO: 80 - protein, 10 aa, Artificial Sequence
  source: /note="Description of Artificial Sequence: Synthetic peptide"
DAWELLAFDI

SEQ ID NO: 81 - protein, 10 aa, Artificial Sequence
  source: /note="Description of Artificial Sequence: Synthetic peptide"
DRWDGDYYSA

SEQ ID NO: 82 - protein, 10 aa, Artificial Sequence
  source: /note="Description of Artificial Sequence: Synthetic peptide"
ESWELTGFDY

SEQ ID NO: 83 - protein, 9 aa, Artificial Sequence
  source: /note="Description of Artificial Sequence: Synthetic peptide"
ERFAGGMDA

SEQ ID NO: 84 - protein, 8 aa, Artificial Sequence
  source: /note="Description of Artificial Sequence: Synthetic peptide"
DSGGAFDI

SEQ ID NO: 85 - protein, 9 aa, Artificial Sequence
  source: /note="Description of Artificial Sequence: Synthetic peptide"
EVFEGGMDV

SEQ ID NO: 86 - protein, 9 aa, Artificial Sequence
  source: /note="Description of Artificial Sequence: Synthetic peptide"
EGYGGNYGN

SEQ ID NO: 87 - protein, 9 aa, Artificial Sequence
  source: /note="Description of Artificial Sequence: Synthetic peptide"
EDFYGDFDY

SEQ ID NO: 88 - protein, 9 aa, Artificial Sequence
  source: /note="Description of Artificial Sequence: Synthetic peptide"
ELSRWGFDY

SEQ ID NO: 89 - protein, 14 aa, Artificial Sequence
  source: /note="Description of Artificial Sequence: Synthetic peptide"
DIFPTMIAGGGFDL

SEQ ID NO: 90 - protein, 10 aa, Artificial Sequence
  source: /note="Description of Artificial Sequence: Synthetic peptide"
GGYSYGSFDY

SEQ ID NO: 91 - protein, 15 aa, Artificial Sequence
  source: /note="Description of Artificial Sequence: Synthetic peptide"
GSFPLVFTIFGVGDV

SEQ ID NO: 92 - protein, 10 aa, Artificial Sequence
  source: /note="Description of Artificial Sequence: Synthetic peptide"
DLDYVRAFDI

SEQ ID NO: 93 - protein, 9 aa, Artificial Sequence
  source: /note="Description of Artificial Sequence: Synthetic peptide"
ESWGGYFDL

SEQ ID NO: 94 - protein, 9 aa, Artificial Sequence
  source: /note="Description of Artificial Sequence: Synthetic peptide"
DRTTYAFDI

SEQ ID NO: 95 - protein, 11 aa, Artificial Sequence
  source: /note="Description of Artificial Sequence: Synthetic peptide"
VHGSGSDGMDV

SEQ ID NO: 96 - protein, 11 aa, Artificial Sequence
  source: /note="Description of Artificial Sequence: Synthetic peptide"
RASQGIDSYLA

SEQ ID NO: 97 - protein, 11 aa, Artificial Sequence
  source: /note="Description of Artificial Sequence: Synthetic peptide"
RASQSISSWLA

SEQ ID NO: 98 - protein, 11 aa, Artificial Sequence
  source: /note="Description of Artificial Sequence: Synthetic peptide"
RASQSISSYLN

SEQ ID NO: 99 - protein, 11 aa, Artificial Sequence
  source: /note="Description of Artificial Sequence: Synthetic peptide"
RASQGISSYLA

SEQ ID NO: 100 - protein, 11 aa, Artificial Sequence
  source: /note="Description of Artificial Sequence: Synthetic peptide"
RASQTISNYLN

SEQ ID NO: 101 - protein, 12 aa, Artificial Sequence
  source: /note="Description of Artificial Sequence: Synthetic peptide"
RASQSVDRNYVT

SEQ ID NO: 102 - protein, 11 aa, Artificial Sequence
  source: /note="Description of Artificial Sequence: Synthetic peptide"
RASQGISQYLA

SEQ ID NO: 103 - protein, 11 aa, Artificial Sequence
  source: /note="Description of Artificial Sequence: Synthetic peptide"
QASQDIGNYLN

SEQ ID NO: 104 - protein, 11 aa, Artificial Sequence
  source: /note="Description of Artificial Sequence: Synthetic peptide"
RASQGIRNDLG

SEQ ID NO: 105 - protein, 11 aa, Artificial Sequence
  source: /note="Description of Artificial Sequence: Synthetic peptide"
RASQIIGNYLA

SEQ ID NO: 106 - protein, 11 aa, Artificial Sequence
  source: /note="Description of Artificial Sequence: Synthetic peptide"
RASQIISSYLN

SEQ ID NO: 107 - protein, 11 aa, Artificial Sequence
  source: /note="Description of Artificial Sequence: Synthetic peptide"
QASQDISNYLN

SEQ ID NO: 108 - protein, 11 aa, Artificial Sequence
  source: /note="Description of Artificial Sequence: Synthetic peptide"
RASQGISNYLA

SEQ ID NO: 109 - protein, 11 aa, Artificial Sequence
  source: /note="Description of Artificial Sequence: Synthetic peptide"
RASQGISNNLN

SEQ ID NO: 110 - protein, 11 aa, Artificial Sequence
  source: /note="Description of Artificial Sequence: Synthetic peptide"
RASQGISNGLS

SEQ ID NO: 111 - protein, 11 aa, Artificial Sequence
  source: /note="Description of Artificial Sequence: Synthetic peptide"
RASQSITGWLA

SEQ ID NO: 112 - protein, 11 aa, Artificial Sequence
  source: /note="Description of Artificial Sequence: Synthetic peptide"
RASQGIRNDLA

SEQ ID NO: 113 - protein, 11 aa, Artificial Sequence
  source: /note="Description of Artificial Sequence: Synthetic peptide"
QASQDISSYLN

SEQ ID NO: 114 - protein, 11 aa, Artificial Sequence
  source: /note="Description of Artificial Sequence: Synthetic peptide"
RASQSITTYLN

SEQ ID NO: 115 - protein, 11 aa, Artificial Sequence
  source: /note="Description of Artificial Sequence: Synthetic peptide"
RASQSVSTWLA

SEQ ID NO: 116 - protein, 11 aa, Artificial Sequence
  source: /note="Description of Artificial Sequence: Synthetic peptide"
RASQSISNWLA

SEQ ID NO: 117 - protein, 11 aa, Artificial Sequence
  source: /note="Description of Artificial Sequence: Synthetic peptide"
QASQGISNYLA

SEQ ID NO: 118 - protein, 12 aa, Artificial Sequence
  source: /note="Description of Artificial Sequence: Synthetic peptide"
RASQSLSSSSLA

SEQ ID NO: 119 - protein, 11 aa, Artificial Sequence
  source: /note="Description of Artificial Sequence: Synthetic peptide"
RASEHIANWLA

SEQ ID NO: 120 - protein, 11 aa, Artificial Sequence
  source: /note="Description of Artificial Sequence: Synthetic peptide"
RASQSVGSWVA

SEQ ID NO: 121 - protein, 11 aa, Artificial Sequence
  source: /note="Description of Artificial Sequence: Synthetic peptide"
RASQSISPWLA

SEQ ID NO: 122 - protein, 11 aa, Artificial Sequence
  source: /note="Description of Artificial Sequence: Synthetic peptide"
RASQGISRYLA

SEQ ID NO: 123 - protein, 12 aa, Artificial Sequence
  source: /note="Description of Artificial Sequence: Synthetic peptide"
RASQTVSSNYLA

SEQ ID NO: 124 - protein, 11 aa, Artificial Sequence
  source: /note="Description of Artificial Sequence: Synthetic peptide"
RSSQGIRNDLS

SEQ ID NO: 125 - protein, 11 aa, Artificial Sequence
  source: /note="Description of Artificial Sequence: Synthetic peptide"
RDSHSITTWLA

SEQ ID NO: 126 - protein, 11 aa, Artificial Sequence
  source: /note="Description of Artificial Sequence: Synthetic peptide"
RASQSISRWLA

SEQ ID NO: 127 - protein, 11 aa, Artificial Sequence
  source: /note="Description of Artificial Sequence: Synthetic peptide"
RASQVIRNDLA

SEQ ID NO: 128 - skipped

SEQ ID NO: 129 - protein, 7 aa, Artificial Sequence
  source: /note="Description of Artificial Sequence: Synthetic peptide"
AASSLQS

SEQ ID NO: 130 - protein, 7 aa, Artificial Sequence
  source: /note="Description of Artificial Sequence: Synthetic peptide"
GASNLQS

SEQ ID NO: 131 - protein, 7 aa, Artificial Sequence
  source: /note="Description of Artificial Sequence: Synthetic peptide"
GASTRAT

SEQ ID NO: 132 - protein, 7 aa, Artificial Sequence
  source: /note="Description of Artificial Sequence: Synthetic peptide"
GASNLHS

SEQ ID NO: 133 - protein, 7 aa, Artificial Sequence
  source: /note="Description of Artificial Sequence: Synthetic peptide"
AASSLES

SEQ ID NO: 134 - protein, 7 aa, Artificial Sequence
  source: /note="Description of Artificial Sequence: Synthetic peptide"
SASNLQS

SEQ ID NO: 135 - protein, 7 aa, Artificial Sequence
  source: /note="Description of Artificial Sequence: Synthetic peptide"
AASTLES

SEQ ID NO: 136 - protein, 7 aa, Artificial Sequence
  source: /note="Description of Artificial Sequence: Synthetic peptide"
HASILET

SEQ ID NO: 137 - protein, 7 aa, Artificial Sequence
  source: /note="Description of Artificial Sequence: Synthetic peptide"
AASTLQS

SEQ ID NO: 138 - protein, 7 aa, Artificial Sequence
  source: /note="Description of Artificial Sequence: Synthetic peptide"
AATTLQS

SEQ ID NO: 139 - protein, 7 aa, Artificial Sequence
  source: /note="Description of Artificial Sequence: Synthetic peptide"
DATHLET

SEQ ID NO: 140 - protein, 7 aa, Artificial Sequence
  source: /note="Description of Artificial Sequence: Synthetic peptide"
AASSLQT

SEQ ID NO: 141 - protein, 7 aa, Artificial Sequence
  source: /note="Description of Artificial Sequence: Synthetic peptide"
AASSLQG

SEQ ID NO: 142 - protein, 7 aa, Artificial Sequence
  source: /note="Description of Artificial Sequence: Synthetic peptide"
AASNLES

SEQ ID NO: 143 - protein, 7 aa, Artificial Sequence
  source: /note="Description of Artificial Sequence: Synthetic peptide"
DVSHLES

SEQ ID NO: 144 - protein, 7 aa, Artificial Sequence
  source: /note="Description of Artificial Sequence: Synthetic peptide"
DASSLQS

SEQ ID NO: 145 - protein, 7 aa, Artificial Sequence
  source: /note="Description of Artificial Sequence: Synthetic peptide"
GVSSLES

SEQ ID NO: 146 - protein, 7 aa, Artificial Sequence
  source: /note="Description of Artificial Sequence: Synthetic peptide"
PASTLQS

SEQ ID NO: 147 - protein, 7 aa, Artificial Sequence
  source: /note="Description of Artificial Sequence: Synthetic peptide"
DASNLET

SEQ ID NO: 148 - protein, 7 aa, Artificial Sequence
  source: /note="Description of Artificial Sequence: Synthetic peptide"
GASTRAS

SEQ ID NO: 149 - protein, 7 aa, Artificial Sequence
  source: /note="Description of Artificial Sequence: Synthetic peptide"
DSSSLQT

SEQ ID NO: 150 - protein, 7 aa, Artificial Sequence
  source: /note="Description of Artificial Sequence: Synthetic peptide"
ATSTLQS

SEQ ID NO: 151 - protein, 7 aa, Artificial Sequence
  source: /note="Description of Artificial Sequence: Synthetic peptide"
LASNSHS

SEQ ID NO: 152 - protein, 9 aa, Artificial Sequence
  source: /note="Description of Artificial Sequence: Synthetic peptide"
QQSYSTPIT

SEQ ID NO: 153 - protein, 9 aa, Artificial Sequence
  source: /note="Description of Artificial Sequence: Synthetic peptide"
QQSYTTPIT

SEQ ID NO: 154 - protein, 9 aa, Artificial Sequence
  source: /note="Description of Artificial Sequence: Synthetic peptide"
QQIFSTPLT

SEQ ID NO: 155 - protein, 9 aa, Artificial Sequence
  source: /note="Description of Artificial Sequence: Synthetic peptide"
QQSYSTPLT

SEQ ID NO: 156 - protein, 9 aa, Artificial Sequence
  source: /note="Description of Artificial Sequence: Synthetic peptide"
QQSYTTPYT

SEQ ID NO: 157 - protein, 9 aa, Artificial Sequence
  source: /note="Description of Artificial Sequence: Synthetic peptide"
QQTFTTPLT

SEQ ID NO: 158 - protein, 9 aa, Artificial Sequence
  source: /note="Description of Artificial Sequence: Synthetic peptide"
QQANSFPFT

SEQ ID NO: 159 - protein, 9 aa, Artificial Sequence
  source: /note="Description of Artificial Sequence: Synthetic peptide"
QQSYTTPYS

SEQ ID NO: 160 - protein, 9 aa, Artificial Sequence
  source: /note="Description of Artificial Sequence: Synthetic peptide"
QQTFITPLT

SEQ ID NO: 161 - protein, 8 aa, Artificial Sequence
  source: /note="Description of Artificial Sequence: Synthetic peptide"
QQSYSTPT

SEQ ID NO: 162 - protein, 9 aa, Artificial Sequence
  source: /note="Description of Artificial Sequence: Synthetic peptide"
QQGFSTPFT

SEQ ID NO: 163 - protein, 9 aa, Artificial Sequence
  source: /note="Description of Artificial Sequence: Synthetic peptide"
QQSFTNPVT

SEQ ID NO: 164 - protein, 9 aa, Artificial Sequence
  source: /note="Description of Artificial Sequence: Synthetic peptide"
QQSYSAPYT

SEQ ID NO: 165 - protein, 9 aa, Artificial Sequence
  source: /note="Description of Artificial Sequence: Synthetic peptide"
QQSYSTPYT

SEQ ID NO: 166 - protein, 9 aa, Artificial Sequence
  source: /note="Description of Artificial Sequence: Synthetic peptide"
QQSHSTPLT

SEQ ID NO: 167 - protein, 9 aa, Artificial Sequence
  source: /note="Description of Artificial Sequence: Synthetic peptide"
QQSYSTPFT

SEQ ID NO: 168 - protein, 9 aa, Artificial Sequence
  source: /note="Description of Artificial Sequence: Synthetic peptide"
QQYGSSPFT

SEQ ID NO: 169 - protein, 9 aa, Artificial Sequence
  source: /note="Description of Artificial Sequence: Synthetic peptide"
QQTYSTPIT

SEQ ID NO: 170 - protein, 9 aa, Artificial Sequence
  source: /note="Description of Artificial Sequence: Synthetic peptide"
QQYYTTPLT

SEQ ID NO: 171 - protein, 9 aa, Artificial Sequence
  source: /note="Description of Artificial Sequence: Synthetic peptide"
QQSFSTPLT

SEQ ID NO: 172 - protein, 9 aa, Artificial Sequence
  source: /note="Description of Artificial Sequence: Synthetic peptide"
QQSYSTPPT

SEQ ID NO: 173 - protein, 9 aa, Artificial Sequence
  source: /note="Description of Artificial Sequence: Synthetic peptide"
LQHNSYPLT

SEQ ID NO: 174 - protein, 9 aa, Artificial Sequence
  source: /note="Description of Artificial Sequence: Synthetic peptide"
QQSYSTPVT

SEQ ID NO: 175 - protein, 9 aa, Artificial Sequence
  source: /note="Description of Artificial Sequence: Synthetic peptide"
QHFYNTQYT

SEQ ID NO: 176 - protein, 10 aa, Artificial Sequence
  source: /note="Description of Artificial Sequence: Synthetic peptide"
QQSLQYPSHF

SEQ ID NO: 177 - protein, 30 aa, Artificial Sequence
  source: /note="Description of Artificial Sequence: Synthetic polypeptide"
QVQLVQSGAEVKKPGASVKVSCKASGGTFS

SEQ ID NO: 178 - protein, 30 aa, Artificial Sequence
  source: /note="Description of Artificial Sequence: Synthetic polypeptide"
QVQLVQSGAEVKKPGASVKVSCKASGYTFT

SEQ ID NO: 179 - protein, 30 aa, Artificial Sequence
  source: /note="Description of Artificial Sequence: Synthetic polypeptide"
QVQLVQSGAEVKKPGASVKVSCKASGYTFN

SEQ ID NO: 180 - protein, 30 aa, Artificial Sequence
  source: /note="Description of Artificial Sequence: Synthetic polypeptide"
QVQLVQSGAEVKKPGASVKVSCKASGNTFT

SEQ ID NO: 181 - protein, 30 aa, Artificial Sequence
  source: /note="Description of Artificial Sequence: Synthetic polypeptide"
QVQLVQSGAEVKKPGASVKVSCKASGHSFT

SEQ ID NO: 182 - protein, 30 aa, Artificial Sequence
  source: /note="Description of Artificial Sequence: Synthetic polypeptide"
QVQLVQSGAEVKKPGASVKVSCKASGYPFT

SEQ ID NO: 183 - protein, 30 aa, Artificial Sequence
  source: /note="Description of Artificial Sequence: Synthetic polypeptide"
QVQLVQSGAEVKKPGASVKVSCKASGYRFT

SEQ ID NO: 184 - protein, 30 aa, Artificial Sequence
  source: /note="Description of Artificial Sequence: Synthetic polypeptide"
QVQLVQSGAEVKKPGSSVKVSCKASGGTFS

SEQ ID NO: 185 - protein, 30 aa, Artificial Sequence
  source: /note="Description of Artificial Sequence: Synthetic polypeptide"
QVQLVQSGAEVKKPGASVKVSCKASGDTFT

SEQ ID NO: 186 - protein, 30 aa, Artificial Sequence
  source: /note="Description of Artificial Sequence: Synthetic polypeptide"
QVQLAQSGAEVKKPGASVKVSCKASGYTFT

SEQ ID NO: 187 - protein, 30 aa, Artificial Sequence
  source: /note="Description of Artificial Sequence: Synthetic polypeptide"
QVQLVQSGAEVKKPGASVKVSCKASGYTFS

SEQ ID NO: 188 - protein, 30 aa, Artificial Sequence
  source: /note="Description of Artificial Sequence: Synthetic polypeptide"
QVQLVQSGAEVKKPGASVKVSCKASGYPFS

SEQ ID NO: 189 - protein, 30 aa, Artificial Sequence
  source: /note="Description of Artificial Sequence: Synthetic polypeptide"
QVQLVQSGAEVKKPGASVKVSCKASGYSFT

SEQ ID NO: 190 - protein, 30 aa, Artificial Sequence
  source: /note="Description of Artificial Sequence: Synthetic polypeptide"
QVQLVQSGAEVKKPGASVKVSCKASGYTFI

SEQ ID NO: 191 - protein, 30 aa, Artificial Sequence
  source: /note="Description of Artificial Sequence: Synthetic polypeptide"
QVQLVQSGAEVKKPGSSVKVSCKASGYTFT

SEQ ID NO: 192 - protein, 14 aa, Artificial Sequence
  source: /note="Description of Artificial Sequence: Synthetic peptide"
WVRQAPGQGLEWMG

SEQ ID NO: 193 - protein, 14 aa, Artificial Sequence
  source: /note="Description of Artificial Sequence: Synthetic peptide"
WVRQAPGQGLEWLG

SEQ ID NO: 194 - protein, 14 aa, Artificial Sequence
  source: /note="Description of Artificial Sequence: Synthetic peptide"
WVRQAPGQGLEWIG

SEQ ID NO: 195 - protein, 14 aa, Artificial Sequence
  source: /note="Description of Artificial Sequence: Synthetic peptide"
WVRQAPGQGLEWVG

SEQ ID NO: 196 - protein, 32 aa, Artificial Sequence
  source: /note="Description of Artificial Sequence: Synthetic polypeptide"
RVTMTRDTSTSTVYMELSSLRSEDTAVYYCAR

SEQ ID NO: 197 - protein, 32 aa, Artificial Sequence
  source: /note="Description of Artificial Sequence: Synthetic polypeptide"
RVTMTRDTSTSTVYMELSSLRSEDTAVYYCAI

SEQ ID NO: 198 - protein, 32 aa, Artificial Sequence
  source: /note="Description of Artificial Sequence: Synthetic polypeptide"
RVTMTRDTSTSTVYMELSSLRSEDTAVYYCTR

SEQ ID NO: 199 - protein, 32 aa, Artificial Sequence
  source: /note="Description of Artificial Sequence: Synthetic polypeptide"
RVTITADESTSTAYMELSSLRSEDTAVYYCAR

SEQ ID NO: 200 - protein, 32 aa, Artificial Sequence
  source: /note="Description of Artificial Sequence: Synthetic polypeptide"
RVTMTRDTSTSTVNMELSSLRSEDTAVYYCAR

SEQ ID NO: 201 - protein, 32 aa, Artificial Sequence
  source: /note="Description of Artificial Sequence: Synthetic polypeptide"
RVTMTRDTSTSTVYMELSSLRSEDTAVYYCAE

SEQ ID NO: 202 - protein, 11 aa, Artificial Sequence
  source: /note="Description of Artificial Sequence: Synthetic peptide"
WGQGTLVTVSS

SEQ ID NO: 203 - protein, 11 aa, Artificial Sequence
  source: /note="Description of Artificial Sequence: Synthetic peptide"
WGQGTTVTVSS

SEQ ID NO: 204 - protein, 11 aa, Artificial Sequence
  source: /note="Description of Artificial Sequence: Synthetic peptide"
WGQGTMVTVSS

SEQ ID NO: 205 - protein, 11 aa, Artificial Sequence
  source: /note="Description of Artificial Sequence: Synthetic peptide"
WGPGTMVTVSS

SEQ ID NO: 206 - protein, 11 aa, Artificial Sequence
  source: /note="Description of Artificial Sequence: Synthetic peptide"
WGRGTLVTVSS

SEQ ID NO: 207 - protein, 23 aa, Artificial Sequence
  source: /note="Description of Artificial Sequence: Synthetic peptide"
DIQMTQSPSSLSASVGDRVTITC

SEQ ID NO: 208 - protein, 23 aa, Artificial Sequence
  source: /note="Description of Artificial Sequence: Synthetic peptide"
EIVMTQSPATLSVSPGERATLSC

SEQ ID NO: 209 - protein, 23 aa, Artificial Sequence
  source: /note="Description of Artificial Sequence: Synthetic peptide"
DIQITHSPSSLSASVGYRLTITC

SEQ ID NO: 210 - protein, 15 aa, Artificial Sequence
  source: /note="Description of Artificial Sequence: Synthetic peptide"
WYQQKPGKAPKLLIY

SEQ ID NO: 211 - protein, 15 aa, Artificial Sequence
  source: /note="Description of Artificial Sequence: Synthetic peptide"
WYQQKPGQAPRLLIY

SEQ ID NO: 212 - protein, 15 aa, Artificial Sequence
  source: /note="Description of Artificial Sequence: Synthetic peptide"
WYHQKPWNAPKLMIY

SEQ ID NO: 213 - protein, 32 aa, Artificial Sequence
  source: /note="Description of Artificial Sequence: Synthetic polypeptide"
GVPSRFSGSGSGTDFTLTISSLQPEDFATYYC

SEQ ID NO: 214 - protein, 32 aa, Artificial Sequence
  source: /note="Description of Artificial Sequence: Synthetic polypeptide"
GIPARFSGSGSGTEFTLTISSLQSEDFAVYYC

SEQ ID NO: 215 - protein, 32 aa, Artificial Sequence
  source: /note="Description of Artificial Sequence: Synthetic polypeptide"
GVPSRFSGSGSGTYFTLTISSLQPEDFATYYC

SEQ ID NO: 216 - protein, 32 aa, Artificial Sequence
  source: /note="Description of Artificial Sequence: Synthetic polypeptide"
GVPSRFSGSGSGTDFTLTISSLQPEDFAPYYC

SEQ ID NO: 217 - protein, 10 aa, Artificial Sequence
  source: /note="Description of Artificial Sequence: Synthetic peptide"
FGGGTKVEIK

SEQ ID NO: 218 - protein, 10 aa, Artificial Sequence
  source: /note="Description of Artificial Sequence: Synthetic peptide"
FGQGTKVEIK

SEQ ID NO: 219 - protein, 10 aa, Artificial Sequence
  source: /note="Description of Artificial Sequence: Synthetic peptide"
FGQGTRLEIK

SEQ ID NO: 220 - protein, 10 aa, Artificial Sequence
  source: /note="Description of Artificial Sequence: Synthetic peptide"
FGGGTKLEIK

SEQ ID NO: 221 - protein, 10 aa, Artificial Sequence
  source: /note="Description of Artificial Sequence: Synthetic peptide"
FGQGTKLEIK

SEQ ID NO: 222 - protein, 10 aa, Artificial Sequence
  source: /note="Description of Artificial Sequence: Synthetic peptide"
FGPGTKVDIK

SEQ ID NO: 223 - protein, 127 aa, Artificial Sequence
  source: /note="Description of Artificial Sequence: Synthetic polypeptide"
QVQLVQSGAEVKKPGASVKVSCKASGGTFSSYAISWVRQAPGQGLEWMGVINPSAGSTDYAQKFQGRVTMTRDTSTSTVYMELSSLRSEDTAVYYCARDLYPYVVVVAAGSYGMDVWGQGTLVTVSS

SEQ ID NO: 224 - protein, 121 aa, Artificial Sequence
  source: /note="Description of Artificial Sequence: Synthetic polypeptide"
QVQLVQSGAEVKKPGASVKVSCKASGYTFTSYYMHWVRQAPGQGLEWMGWMNPNSDIAGYAQKFQGRVTMTRDTSTSTVYMELSSLRSEDTAVYYCAIPSIVGAYDAFDIWGQGTLVTVSS

SEQ ID NO: 225 - protein, 118 aa, Artificial Sequence
  source: /note="Description of Artificial Sequence: Synthetic polypeptide"
QVQLVQSGAEVKKPGASVKVSCKASGYTFTRHLLHWVRQAPGQGLEWMGWISPQHGVRNYAQKFQGRVTMTRDTSTSTVYMELSSLRSEDTAVYYCARESVEGYFDLWGQGTLVTVSS

SEQ ID NO: 226 - protein, 120 aa, Artificial Sequence
  source: /note="Description of Artificial Sequence: Synthetic polypeptide"
QVQLVQSGAEVKKPGASVKVSCKASGYTFTSHHMHWVRQAPGQGLEWMGWVSPSHGLTGYAQKFQGRVTMTRDTSTSTVYMELSSLRSEDTAVYYCARDNWNVHDAFDIWGQGTLVTVSS

SEQ ID NO: 227 - protein, 117 aa, Artificial Sequence
  source: /note="Description of Artificial Sequence: Synthetic polypeptide"
QVQLVQSGAEVKKPGASVKVSCKASGYTFNRFMHWVRQAPGQGLEWMGWMSLNSGLTGYAQKFQGRVTMTRDTSTSTVYMELSSLRSEDTAVYYCTRGTYNDAFDIWGQGTLVTVSS

SEQ ID NO: 228 - protein, 120 aa, Artificial Sequence
  source: /note="Description of Artificial Sequence: Synthetic polypeptide"
QVQLVQSGAEVKKPGASVKVSCKASGYTFTSYYIHWVRQAPGQGLEWMGWMKPSSGTTGYAQKFQGRVTMTRDTSTSTVYMELSSLRSEDTAVYYCAREQWLVNDAFDIWGQGTLVTVSS

SEQ ID NO: 229 - protein, 120 aa, Artificial Sequence; identical to SEQ ID NO: 228
  source: /note="Description of Artificial Sequence: Synthetic polypeptide"

SEQ ID NO: 230 - protein, 123 aa, Artificial Sequence
  source: /note="Description of Artificial Sequence: Synthetic polypeptide"
QVQLVQSGAEVKKPGASVKVSCKASGNTFTSYYMHWVRQAPGQGLEWMGGIDPNSGGTNYAQKFQGRVTMTRDTSTSTVYMELSSLRSEDTAVYYCARSMFPTIFGDNAFDIWGQGTLVTVSS

SEQ ID NO: 231 - protein, 123 aa, Artificial Sequence
  source: /note="Description of Artificial Sequence: Synthetic polypeptide"
QVQLVQSGAEVKKPGASVKVSCKASGHSFTHYYMHWVRQAPGQGLEWMGWMNPDSGSTGYAQKFQGRVTMTRDTSTSTVYMELSSLRSEDTAVYYCARALFPYPFYYYYMDVWGQGTLVTVSS

SEQ ID NO: 232 - protein, 116 aa, Artificial Sequence
  source: /note="Description of Artificial Sequence: Synthetic polypeptide"
QVQLVQSGAEVKKPGASVKVSCKASGYTFTGYYMHWVRQAPGQGLEWIGWMSLNSGLTGYAQKFQGRVTMTRDTSTSTVYMELSSLRSEDTAVYYCARDRGWFDPWGQGTLVTVSS

SEQ ID NO: 233 - protein, 122 aa, Artificial Sequence
  source: /note="Description of Artificial Sequence: Synthetic polypeptide"
QVQLVQSGAEVKKPGASVKVSCKASGYTFTNYYIHWVRQAPGQGLEWLGWMNPNGDVAGYADSFQGRVTMTRDTSTSTVYMELSSLRSEDTAVYYCAIDSSGWMRNDAFDIWGQGTLVTVSS

SEQ ID NO: 234 - protein, 119 aa, Artificial Sequence
  source: /note="Description of Artificial Sequence: Synthetic polypeptide"
QVQLVQSGAEVKKPGASVKVSCKASGGTFSNYMYHWVRQAPGQGLEWMGWISTYHGSTNYAQKFQGRVTMTRDTSTSTVYMELSSLRSEDTAVYYCARDARGYSGYDLWGQGTLVTVSS

SEQ ID NO: 235 - protein, 118 aa, Artificial Sequence
  source: /note="Description of Artificial Sequence: Synthetic polypeptide"
QVQLVQSGAEVKKPGASVKVSCKASGYPFTSYYMHWVRQAPGQGLEWMGWMNPNSDIAGYAQKFQGRVTMTRDTSTSTVYMELSSLRSEDTAVYYCAREGRHGEYLYWGQGTLVTVSS

SEQ ID NO: 236 - protein, 120 aa, Artificial Sequence
  source: /note="Description of Artificial Sequence: Synthetic polypeptide"
QVQLVQSGAEVKKPGASVKVSCKASGYRFTTYYVHWVRQAPGQGLEWMGWMNPNTVYTGSAQKFQGRVTMTRDTSTSTVYMELSSLRSEDTAVYYCAREGWGSSGYFDYWGQGTLVTVSS

SEQ ID NO: 237 - protein, 124 aa, Artificial Sequence
  source: /note="Description of Artificial Sequence: Synthetic polypeptide"
QVQLVQSGAEVKKPGSSVKVSCKASGGTFSSYALSWVRQAPGQGLEWMGRIIPAVGSVTYAQKFQGRVTITADESTSTAYMELSSLRSEDTAVYYCARHLFPTVFDDYYGMDVWGQGTLVTVSS

SEQ ID NO: 238 - protein, 119 aa, Artificial Sequence
  source: /note="Description of Artificial Sequence: Synthetic polypeptide"
QVQLVQSGAEVKKPGSSVKVSCKASGGTFSSYAISWVRQAPGQGLEWMGGIIPIFGTANYAQKFQGRVTITADESTSTAYMELSSLRSEDTAVYYCARGGYSYGSFQHWGQGTLVTVSS

SEQ ID NO: 239 - protein, 119 aa, Artificial Sequence
  source: /note="Description of Artificial Sequence: Synthetic polypeptide"
QVQLVQSGAEVKKPGASVKVSCKASGDTFTRHYVHWVRQAPGQGLEWMGWMSPSSGITGYAQKFQGRVTMTRDTSTSTVYMELSSLRSEDTAVYYCARVRWSSDAFDIWGQGTLVTVSS

SEQ ID NO: 240 - protein, 118 aa, Artificial Sequence
  source: /note="Description of Artificial Sequence: Synthetic polypeptide"
QVQLVQSGAEVKKPGASVKVSCKASGYTFTSYYMHWVRQAPGQGLEWVGWMTPSTGNAGYAQKFQGRVTMTRDTSTSTVYMELSSLRSEDTAVYYCAREEWLGHFQHWGQGTLVTVSS

SEQ ID NO: 241 - protein, 118 aa, Artificial Sequence
  source: /note="Description of Artificial Sequence: Synthetic polypeptide"
QVQLVQSGAEVKKPGASVKVSCKASGYTFTSHYMHWVRQAPGQGLEWMGWMNPNSGNTGYAQKFQGRVTMTRDTSTSTVYMELSSLRSEDTAVYYCARERFLGGMDVWGQGTTVTVSS

SEQ ID NO: 242 - protein, 118 aa, Artificial Sequence
  source: /note="Description of Artificial Sequence: Synthetic polypeptide"
QVQLVQSGAEVKKPGASVKVSCKASGYTFTDYYMHWVRQAPGQGLEWMGWMHPNSGHTGYAQKFQGRVTMTRDTSTSTVNMELSSLRSEDTAVYYCAREEWLGHFQHWGQGTLVTVSS

SEQ ID NO: 243 - protein, 118 aa, Artificial Sequence
  source: /note="Description of Artificial Sequence: Synthetic polypeptide"
QVQLVQSGAEVKKPGASVKVSCKASGYTFTSHYMHWVRQAPGQGLEWMGWMNPNSGHTGNAQKFQGRVTMTRDTSTSTVYMELSSLRSEDTAVYYCARGNWVDAFDIWGQGTMVTVSS

SEQ ID NO: 244 - protein, 120 aa, Artificial Sequence
  source: /note="Description of Artificial Sequence: Synthetic polypeptide"
QVQLVQSGAEVKKPGASVKVSCKASGYTFTGYTLHWVRQAPGQGLEWMGWIDPNSGVTSSAQKFQGRVTMTRDTSTSTVYMELSSLRSEDTAVYYCARESEVMMAYFQHWGQGTLVTVSS

SEQ ID NO: 245 - protein, 118 aa, Artificial Sequence
  source: /note="Description of Artificial Sequence: Synthetic polypeptide"
QVQLVQSGAEVKKPGASVKVSCKASGYTFTGYYMHWVRQAPGQGLEWMGWISPNSGVTDFTQKFQGRVTMTRDTSTSTVYMELSSLRSEDTAVYYCARESWSGEFDYWGQGTLVTVSS

SEQ ID NO: 246 - protein, 118 aa, Artificial Sequence
  source: /note="Description of Artificial Sequence: Synthetic polypeptide"
QVQLVQSGAEVKKPGASVKVSCKASGDTFTNHYMHWVRQAPGQGLEWMGWMNPNSGHTGYAQRFQGRVTMTRDTSTSTVYMELSSLRSEDTAVYYCAREAVAGPMDVWGQGTTVTVSS

SEQ ID NO: 247 - protein, 119 aa, Artificial Sequence
  source: /note="Description of Artificial Sequence: Synthetic polypeptide"
QVQLVQSGAEVKKPGASVKVSCKASGYTFTGYYMHWVRQAPGQGLEWMGWMNPNSDIAGYAQKFQGRVTMTRDTSTSTVYMELSSLRSEDTAVYYCARDAWELLAFDIWGQGTLVTVSS

SEQ ID NO: 248 - protein, 119 aa, Artificial Sequence
  source: /note="Description of Artificial Sequence: Synthetic polypeptide"
QVQLAQSGAEVKKPGASVKVSCKASGYTFTNHYMHWVRQAPGQGLEWMGWMNPNSGNTGYAQKFQGRVTMTRDTSTSTVYMELSSLRSEDTAVYYCARDRWDGDYYSAWGQGTLVTVSS

SEQ ID NO: 249 - protein, 119 aa, Artificial Sequence
  source: /note="Description of Artificial Sequence: Synthetic polypeptide"
QVQLVQSGAEVKKPGASVKVSCKASGYTFTNYYIHWVRQAPGQGLEWMGWMSPNGGNTGYAQKFQGRVTMTRDTSTSTVYMELSSLRSEDTAVYYCARESWELTGFDYWGQGTLVTVSS

SEQ ID NO: 250 - protein, 118 aa, Artificial Sequence
  source: /note="Description of Artificial Sequence: Synthetic polypeptide"
QVQLVQSGAEVKKPGASVKVSCKASGYTFTSYYMHWVRQAPGQGLEWMGWMNPNSGNTGYAQKFQGRVTMTRDTSTSTVYMELSSLRSEDTAVYYCARERFAGGMDAWGQGTTVTVSS

SEQ ID NO: 251 - protein, 117 aa, Artificial Sequence
  source: /note="Description of Artificial Sequence: Synthetic polypeptide"
QVQLVQSGAEVKKPGASVKVSCKASGYTFSNSYMHWVRQAPGQGLEWMGWMDPSSGYTGSAHKFQGRVTMTRDTSTSTVYMELSSLRSEDTAVYYCAEDSGGAFDIWGQGTMVTVSS

SEQ ID NO: 252 - protein, 118 aa, Artificial Sequence
  source: /note="Description of Artificial Sequence: Synthetic polypeptide"
QVQLVQSGAEVKKPGASVKVSCKASGYPFSTYYMHWVRQAPGQGLEWMGWMNPHSADTGYAEKFQGRVTMTRDTSTSTVYMELSSLRSEDTAVYYCAREVFEGGMDVWGQGTTVTVSS

SEQ ID NO: 253 - protein, 118 aa, Artificial Sequence
  source: /note="Description of Artificial Sequence: Synthetic polypeptide"
QVQLVQSGAEVKKPGASVKVSCKASGYTFTSYYMHWVRQAPGQGLEWMGWLTPSTGHAGYAQKFQGRVTMTRDTSTSTVYMELSSLRSEDTAVYYCAREGYGGNYGNWGQGTLVTVSS

SEQ ID NO: 254 - protein, 118 aa, Artificial Sequence
  source: /note="Description of Artificial Sequence: Synthetic polypeptide"
QVQLVQSGAEVKKPGASVKVSCKASGYTFTSYYMHWVRQAPGQGLEWMGWMNPNSGHTGYAQKFQGRVTMTRDTSTSTVYMELSSLRSEDTAVYYCAREDFYGDFDYWGQGTLVTVSS

SEQ ID NO: 255 - protein, 118 aa, Artificial Sequence
  source: /note="Description of Artificial Sequence: Synthetic polypeptide"
QVQLVQSGAEVKKPGASVKVSCKASGYTFTRHFIHWVRQAPGQGLEWMGWIDPNSGVTSSAQKFQGRVTMTRDTSTSTVYMELSSLRSEDTAVYYCARELSRWGFDYWGPGTMVTVSS

SEQ ID NO: 256 - protein, 118 aa, Artificial Sequence
  source: /note="Description of Artificial Sequence: Synthetic polypeptide"
QVQLVQSGAEVKKPGASVKVSCKASGYTFTRHLLHWVRQAPGQGLEWMGWISPQHGVRNYAHKFQGRVTMTRDTSTSTVYMELSSLRSEDTAVYYCARESVEGYFDLWGRGTLVTVSS

SEQ ID NO: 257 - protein, 123 aa, Artificial Sequence
  source: /note="Description of Artificial Sequence: Synthetic polypeptide"
QVQLVQSGAEVKKPGASVKVSCKASGYPFSSYYMHWVRQAPGQGLEWMGMINPSGGSTSYAQKFQGRVTMTRDTSTSTVYMELSSLRSEDTAVYYCARDIFPTMIAGGGFDLWGRGTLVTVSS

SEQ ID NO: 258 - protein, 119 aa, Artificial Sequence
  source: /note="Description of Artificial Sequence: Synthetic polypeptide"
QVQLVQSGAEVKKPGSSVKVSCKASGGTFSTFGISWVRQAPGQGLEWMGGIIPIFGTANYAQKFQGRVTITADESTSTAYMELSSLRSEDTAVYYCARGGYSYGSFDYWGQGTLVTVSS

SEQ ID NO: 259 - protein, 124 aa, Artificial Sequence
  source: /note="Description of Artificial Sequence: Synthetic polypeptide"
QVQLVQSGAEVKKPGASVKVSCKASGYTFTSYGINWVRQAPGQGLEWMGWMNPNSGNTGYAQKFQGRVTMTRDTSTSTVYMELSSLRSEDTAVYYCARGSFPLVFTIFGVGDVWGQGTMVTVSS

SEQ ID NO: 260 - protein, 119 aa, Artificial Sequence
  source: /note="Description of Artificial Sequence: Synthetic polypeptide"
QVQLVQSGAEVKKPGASVKVSCKASGYTFTSYYMHWVRQAPGQGLEWMGWISPRSGVTSYAQKFQGRVTMTRDTSTSTVYMELSSLRSEDTAVYYCARDLDYVRAFDIWGQGTTVTVSS

SEQ ID NO: 261 - protein, 118 aa, Artificial Sequence
  source: /note="Description of Artificial Sequence: Synthetic polypeptide"
QVQLVQSGAEVKKPGASVKVSCKASGYSFTSYYMHWVRQAPGQGLEWMGWMDPNSGNTGYAQKFQGRVTMTRDTSTSTVYMELSSLRSEDTAVYYCARESWGGYFDLWGRGTLVTVSS

SEQ ID NO: 262 - protein, 118 aa, Artificial Sequence
  source: /note="Description of Artificial Sequence: Synthetic polypeptide"
QVQLVQSGAEVKKPGASVKVSCKASGYTFINHYVHWVRQAPGQGLEWMGWMNPTGGITGYAQKFQGRVTMTRDTSTSTVYMELSSLRSEDTAVYYCARDRTTYAFDIWGQGTMVTVSS

SEQ ID NO: 263 - protein, 118 aa, Artificial Sequence; identical to SEQ ID NO: 243
  source: /note="Description of Artificial Sequence: Synthetic polypeptide"

SEQ ID NO: 264 - protein, 120 aa, Artificial Sequence
  source: /note="Description of Artificial Sequence: Synthetic polypeptide"
QVQLVQSGAEVKKPGSSVKVSCKASGYTFTRHLLHWVRQAPGQGLEWMGWVSPIHGLTGYAPRFQGRVTITADESTSTAYMELSSLRSEDTAVYYCARVHGSGSDGMDVWGQGTTVTVSS

SEQ ID NO: 265 - protein, 107 aa, Artificial Sequence
  source: /note="Description of Artificial Sequence: Synthetic polypeptide"
DIQMTQSPSSLSASVGDRVTITCRASQGIDSYLAWYQQKPGKAPKLLIYAASSLQSGVPSRFSGSGSGTDFTLTISSLQPEDFATYYCQQSYSTPITFGGGTKVEIK

SEQ ID NO: 266 - protein, 107 aa, Artificial Sequence
  source: /note="Description of Artificial Sequence: Synthetic polypeptide"
DIQMTQSPSSLSASVGDRVTITCRASQSISSWLAWYQQKPGKAPKLLIYAASSLQSGVPSRFSGSGSGTDFTLTISSLQPEDFATYYCQQSYTTPITFGGGTKVEIK

SEQ ID NO: 267 - protein, 107 aa, Artificial Sequence
  source: /note="Description of Artificial Sequence: Synthetic polypeptide"
DIQMTQSPSSLSASVGDRVTITCRASQSISSYLNWYQQKPGKAPKLLIYAASSLQSGVPSRFSGSGSGTDFTLTISSLQPEDFATYYCQQIFSTPLTFGGGTKVEIK

SEQ ID NO: 268 - protein, 107 aa, Artificial Sequence
  source: /note="Description of Artificial Sequence: Synthetic polypeptide"
DIQMTQSPSSLSASVGDRVTITCRASQGISSYLAWYQQKPGKAPKLLIYGASNLQSGVPSRFSGSGSGTDFTLTISSLQPEDFATYYCQQSYSTPLTFGGGTKVEIK

SEQ ID NO: 269 - protein, 107 aa, Artificial Sequence
  source: /note="Description of Artificial Sequence: Synthetic polypeptide"
DIQMTQSPSSLSASVGDRVTITCRASQTISNYLNWYQQKPGKAPKLLIYAASSLQSGVPSRFSGSGSGTDFTLTISSLQPEDFATYYCQQSYTTPITFGGGTKVEIK

SEQ ID NO: 270 - protein, 108 aa, Artificial Sequence
  source: /note="Description of Artificial Sequence: Synthetic polypeptide"
EIVMTQSPATLSVSPGERATLSCRASQSVDRNYVTWYQQKPGQAPRLLIYGASTRATGIPARFSGSGSGTEFTLTISSLQSEDFAVYYCQQSYTTPYTFGQGTKVEIK

SEQ ID NO: 271 - protein, 107 aa, Artificial Sequence
  source: /note="Description of Artificial Sequence: Synthetic polypeptide"
DIQMTQSPSSLSASVGDRVTITCRASQGISQYLAWYQQKPGKAPKLLIYGASNLHSGVPSRFSGSGSGTDFTLTISSLQPEDFATYYCQQTFTTPLTFGGGTKVEIK

SEQ ID NO: 272 - protein, 107 aa, Artificial Sequence
  source: /note="Description of Artificial Sequence: Synthetic polypeptide"
DIQMTQSPSSLSASVGDRVTITCQASQDIGNYLNWYQQKPGKAPKLLIYAASSLESGVPSRFSGSGSGTDFTLTISSLQPEDFATYYCQQSYSTPLTFGGGTKVEIK

SEQ ID NO: 273 - protein, 107 aa, Artificial Sequence
  source: /note="Description of Artificial Sequence: Synthetic polypeptide"
DIQMTQSPSSLSASVGDRVTITCRASQGIRNDLGWYQQKPGKAPKLLIYSASNLQSGVPSRFSGSGSGTDFTLTISSLQPEDFATYYCQQANSFPFTFGGGTKVEIK

SEQ ID NO: 274 - protein, 107 aa, Artificial Sequence
  source: /note="Description of Artificial Sequence: Synthetic polypeptide"
DIQMTQSPSSLSASVGDRVTITCRASQSISSWLAWYQQKPGKAPKLLIYAASTLESGVPSRFSGSGSGTDFTLTISSLQPEDFATYYCQQSYTTPYSFGGGTKVEIK

SEQ ID NO: 275 - protein, 107 aa, Artificial Sequence
  source: /note="Description of Artificial Sequence: Synthetic polypeptide"
DIQMTQSPSSLSASVGDRVTITCRASQGISQYLAWYQQKPGKAPKLLIYGASNLHSGVPSRFSGSGSGTDFTLTISSLQPEDFATYYCQQTFITPLTFGGGTKVEIK

SEQ ID NO: 276 - protein, 106 aa, Artificial Sequence
  source: /note="Description of Artificial Sequence: Synthetic polypeptide"
DIQMTQSPSSLSASVGDRVTITCRASQIIGNYLAWYQQKPGKAPKLLIYHASILETGVPSRFSGSGSGTDFTLTISSLQPEDFATYYCQQSYSTPTFGGGTKVEIK

SEQ ID NO: 277 - protein, 107 aa, Artificial Sequence
  source: /note="Description of Artificial Sequence: Synthetic polypeptide"
DIQMTQSPSSLSASVGDRVTITCRASQIISSYLNWYQQKPGKAPKLLIYAASSLQSGVPSRFSGSGSGTDFTLTISSLQPEDFATYYCQQGFSTPFTFGGGTKVEIK

SEQ ID NO: 278 - protein, 107 aa, Artificial Sequence
  source: /note="Description of Artificial Sequence: Synthetic polypeptide"
DIQMTQSPSSLSASVGDRVTITCQASQDISNYLNWYQQKPGKAPKLLIYAASSLQSGVPSRFSGSGSGTDFTLTISSLQPEDFATYYCQQSFTNPVTFGGGTKVEIK

SEQ ID NO: 279 - protein, 107 aa, Artificial Sequence
  source: /note="Description of Artificial Sequence: Synthetic polypeptide"
DIQMTQSPSSLSASVGDRVTITCRASQGISNYLAWYQQKPGKAPKLLIYAASTLQSGVPSRFSGSGSGTDFTLTISSLQPEDFATYYCQQSYSAPYTFGGGTKVEIK

SEQ ID NO: 280 - protein, 107 aa, Artificial Sequence
  source: /note="Description of Artificial Sequence: Synthetic polypeptide"
DIQMTQSPSSLSASVGDRVTITCRASQGISNNLNWYQQKPGKAPKLLIYAATTLQSGVPSRFSGSGSGTDFTLTISSLQPEDFATYYCQQSYSTPYTFGGGTKVEIK

SEQ ID NO: 281 - protein, 107 aa, Artificial Sequence [sequence omitted]

SEQ ID NO: 282 - protein, 107 aa, Artificial Sequence
  source: /note="Description of Artificial Sequence: Synthetic polypeptide"
DIQMTQSPSSLSASVGDRVTITCRASQGISNGLSWYQQKPGKAPKLLIYAASTLQSGVPSRFSGSGSGTDFTLTISSLQPEDFATYYCQQSHSTPLTFGGGTKVEIK

SEQ ID NO: 283 - protein, 107 aa, Artificial Sequence
  source: /note="Description of Artificial Sequence: Synthetic polypeptide"
DIQMTQSPSSLSASVGDRVTITCRASQSITGWLAWYQQKPGKAPKLLIYAASSLQSGVPSRFSGSGSGTDFTLTISSLQPEDFATYYCQQSYSTPYTFGQGTKVEIK

SEQ ID NO: 284 - protein, 107 aa, Artificial Sequence
  source: /note="Description of Artificial Sequence: Synthetic polypeptide"
DIQMTQSPSSLSASVGDRVTITCRASQSISSWLAWYQQKPGKAPKLLIYDATHLETGVPSRFSGSGSGTDFTLTISSLQPEDFATYYCQQSYSTPITFGQGTRLEIK

SEQ ID NO: 285 - protein, 107 aa, Artificial Sequence
  source: /note="Description of Artificial Sequence: Synthetic polypeptide"
DIQMTQSPSSLSASVGDRVTITCRASQGIRNDLAWYQQKPGKAPKLLIYAASTLQSGVPSRFSGSGSGTDFTLTISSLQPEDFATYYCQQSYSTPLTFGGGTKVEIK

SEQ ID NO: 286 - protein, 107 aa, Artificial Sequence
  source: /note="Description of Artificial Sequence: Synthetic polypeptide"
DIQMTQSPSSLSASVGDRVTITCQASQDISSYLNWYQQKPGKAPKLLIYAASSLQTGVPSRFSGSGSGTDFTLTISSLQPEDFATYYCQQSYSTPYTFGQGTKLEIK

SEQ ID NO: 287 - protein, 107 aa, Artificial Sequence
  source: /note="Description of Artificial Sequence: Synthetic polypeptide"
DIQMTQSPSSLSASVGDRVTITCRASQSITTYLNWYQQKPGKAPKLLIYAASSLQGGVPSRFSGSGSGTDFTLTISSLQPEDFATYYCQQSYSTPYTFGQGTKVEIK

SEQ ID NO: 288 - protein, 107 aa, Artificial Sequence
  source: /note="Description of Artificial Sequence: Synthetic polypeptide"
DIQMTQSPSSLSASVGDRVTITCRASQSISSYLNWYQQKPGKAPKLLIYAASSLQSGVPSRFSGSGSGTDFTLTISSLQPEDFATYYCQQSYSTPLTFGGGTKLEIK

SEQ ID NO: 289 - protein, 107 aa, Artificial Sequence
  source: /note="Description of Artificial Sequence: Synthetic polypeptide"
DIQMTQSPSSLSASVGDRVTITCRASQSVSTWLAWYQQKPGKAPKLLIYAASNLESGVPSRFSGSGSGTDFTLTISSLQPEDFATYYCQQSYSTPYTFGQGTKLEIK

SEQ ID NO: 290 - protein, 107 aa, Artificial Sequence
  source: /note="Description of Artificial Sequence: Synthetic polypeptide"
DIQMTQSPSSLSASVGDRVTITCRASQSISNWLAWYQQKPGKAPKLLIYDVSHLESGVPSRFSGSGSGTDFTLTISSLQPEDFATYYCQQSYSTPFTFGPGTKVDIK

SEQ ID NO: 291 - protein, 107 aa, Artificial Sequence
  source: /note="Description of Artificial Sequence: Synthetic polypeptide"
DIQMTQSPSSLSASVGDRVTITCQASQGISNYLAWYQQKPGKAPKLLIYDASSLQSGVPSRFSGSGSGTDFTLTISSLQPEDFATYYCQQSYSTPLTFGGGTKVEIK

SEQ ID NO: 292 - protein, 108 aa, Artificial Sequence
  source: /note="Description of Artificial Sequence: Synthetic polypeptide"
EIVMTQSPATLSVSPGERATLSCRASQSLSSSSLAWYQQKPGQAPRLLIYGASTRATGIPARFSGSGSGTEFTLTISSLQSEDFAVYYCQQYGSSPFTFGPGTKVDIK

SEQ ID NO: 293 - protein, 107 aa, Artificial Sequence
  source: /note="Description of Artificial Sequence: Synthetic polypeptide"
DIQMTQSPSSLSASVGDRVTITCRASEHIANWLAWYQQKPGKAPKLLIYGVSSLESGVPSRFSGSGSGTDFTLTISSLQPEDFATYYCQQSYSTPYTFGQGTKLEIK

SEQ ID NO: 294 - protein, 107 aa, Artificial Sequence
  source: /note="Description of Artificial Sequence: Synthetic polypeptide"
DIQMTQSPSSLSASVGDRVTITCRASQSVGSWVAWYQQKPGKAPKLLIYPASTLQSGVPSRFSGSGSGTDFTLTISSLQPEDFATYYCQQSYSTPLTFGGGTKVEIK

SEQ ID NO: 295 - protein, 107 aa, Artificial Sequence
  source: /note="Description of Artificial Sequence: Synthetic polypeptide"
DIQMTQSPSSLSASVGDRVTITCRASQSISPWLAWYQQKPGKAPKLLIYDASNLETGVPSRFSGSGSGTDFTLTISSLQPEDFATYYCQQTYSTPITFGQGTRLEIK

SEQ ID NO: 296 - protein, 107 aa, Artificial Sequence
  source: /note="Description of Artificial Sequence: Synthetic polypeptide"
DIQMTQSPSSLSASVGDRVTITCRASQGISRYLAWYQQKPGKAPKLLIYAASTLQSGVPSRFSGSGSGTDFTLTISSLQPEDFATYYCQQSYSTPLTFGQGTKVEIK

SEQ ID NO: 297 - protein, 108 aa, Artificial Sequence
  source: /note="Description of Artificial Sequence: Synthetic polypeptide"
EIVMTQSPATLSVSPGERATLSCRASQTVSSNYLAWYQQKPGQAPRLLIYGASTRASGIPARFSGSGSGTEFTLTISSLQSEDFAVYYCQQYYTTPLTFGGGTKVEIK

SEQ ID NO: 298 - protein, 107 aa, Artificial Sequence
  source: /note="Description of Artificial Sequence: Synthetic polypeptide"
DIQMTQSPSSLSASVGDRVTITCRASQSISSYLNWYQQKPGKAPKLLIYAASSLQSGVPSRFSGSGSGTDFTLTISSLQPEDFATYYCQQSFSTPLTFGQGTRLEIK

SEQ ID NO: 299 - protein, 107 aa, Artificial Sequence
  source: /note="Description of Artificial Sequence: Synthetic polypeptide"
DIQMTQSPSSLSASVGDRVTITCRASQSISSWLAWYQQKPGKAPKLLIYDASNLETGVPSRFSGSGSGTDFTLTISSLQPEDFATYYCQQSYSTPPTFGQGTKVEIK

SEQ ID NO: 300 - protein, 107 aa, Artificial Sequence
  source: /note="Description of Artificial Sequence: Synthetic polypeptide"
DIQMTQSPSSLSASVGDRVTITCRASQGISNNLNWYQQKPGKAPKLLIYATSTLQSGVPSRFSGSGSGTDFTLTISSLQPEDFATYYCQQSYSTPYTFGQGTKVEIK

SEQ ID NO: 301 - protein, 107 aa, Artificial Sequence
  source: /note="Description of Artificial Sequence: Synthetic polypeptide"
DIQMTQSPSSLSASVGDRVTITCRSSQGIRNDLSWYQQKPGKAPKLLIYLASNSHSGVPSRFSGSGSGTDFTLTISSLQPEDFATYYCLQHNSYPLTFGGGTKVEIK

SEQ ID NO: 302 - protein, 107 aa, Artificial Sequence
  source: /note="Description of Artificial Sequence: Synthetic polypeptide"
DIQMTQSPSSLSASVGDRVTITCRASQSISRWLAWYQQKPGKAPKLLIYAASSLQSGVPSRFSGSGSGTDFTLTISSLQPEDFATYYCQQSYSTPYTFGQGTKLEIK

SEQ ID NO: 303 - protein, 107 aa, Artificial Sequence
  source: /note="Description of Artificial Sequence: Synthetic polypeptide"
DIQMTQSPSSLSASVGDRVTITCRASQSISSWLAWYQQKPGKAPKLLIYDSSSLQTGVPSRFSGSGSGTDFTLTISSLQPEDFATYYCQQSYSTPVTFGQGTKVEIK

SEQ ID NO: 304 - protein, 107 aa, Artificial Sequence
  source: /note="Description of Artificial Sequence: Synthetic polypeptide"
DIQITHSPSSLSASVGYRLTITCRDSHSITTWLAWYHQKPWNAPKLMIYAASNLESGVPSRFSGSGSGTYFTLTISSLQPEDFATYYCQHFYNTQYTFGQGTKVEIK

SEQ ID NO: 305 - protein, 108 aa, Artificial Sequence
  source: /note="Description of Artificial Sequence: Synthetic polypeptide"
DIQMTQSPSSLSASVGDRVTITCRASQVIRNDLAWYQQKPGKAPKLLIYAASTLQSGVPSRFSGSGSGTDFTLTISSLQPEDFATYYCQQSLQYPSHFFGQGTKVEIK

SEQ ID NO: 306 - protein, 107 aa, Artificial Sequence
  source: /note="Description of Artificial Sequence: Synthetic polypeptide"
DIQMTQSPSSLSASVGDRVTITCRASQSISRYLNWYQQKPGKAPKLLIYAASTLQSGVPSRFSGSGSGTDFTLTISSLQPEDFAPYYCQQSYSTPLTFGPGTKVDIK

SEQ ID NO: 307 - protein, 290 aa, Artificial Sequence
  source: /note="Description of Artificial Sequence: Synthetic polypeptide"
MRIFAVFIFMTYWHLLNAFTVTVPKDLYVVEYGSNMTIECKFPVEKQLDLAALIVYWEMEDKNIIQFVHGEEDLKVQHSSYRQRARLLKDQLSLGNAALQITDVKLQDAGVYRCMISYGGADYKRITVKVNAPYNKINQRILVVDPVTSEHELTCQAEGYPKAEVIWTSSDHQVLSGKTTTTNSKREEKLFNVTSTLRINTTTNEIFYCTFRRLDPEENHTAELVIPELPLAHPPNERTHLVILGAILLCLGVALTFIFRLRKGRMMDVKKCGIQDTNSKKQSDTHLEET

SEQ ID NO: 308 - protein, 5 aa, Artificial Sequence
  source: /note="Description of Artificial Sequence: Synthetic peptide"
SDYMH

SEQ ID NO: 309 - protein, 5 aa, Artificial Sequence
  source: /note="Description of Artificial Sequence: Synthetic peptide"
GYYMH

SEQ ID NO: 310 - protein, 5 aa, Artificial Sequence
  source: /note="Description of Artificial Sequence: Synthetic peptide"
SYYMH

SEQ ID NO: 311 - protein, 5 aa, Artificial Sequence
  source: /note="Description of Artificial Sequence: Synthetic peptide"
GYYIH

SEQ ID NO: 312 - protein, 5 aa, Artificial Sequence
  source: /note="Description of Artificial Sequence: Synthetic peptide"
THYMH

SEQ ID NO: 313 - protein, 5 aa, Artificial Sequence
  source: /note="Description of Artificial Sequence: Synthetic peptide"
SHDIN

SEQ ID NO: 314 - protein, 5 aa, Artificial Sequence
  source: /note="Description of Artificial Sequence: Synthetic peptide"
DHYLH

SEQ ID NO: 315 - protein, 5 aa, Artificial Sequence
  source: /note="Description of Artificial Sequence: Synthetic peptide"
NYYMH

SEQ ID NO: 316 - protein, 5 aa, Artificial Sequence
  source: /note="Description of Artificial Sequence: Synthetic peptide"
AYYVH

SEQ ID NO: 317 - protein, 5 aa, Artificial Sequence
  source: /note="Description of Artificial Sequence: Synthetic peptide"
RHYVH

SEQ ID NO: 318 - protein, 4 aa, Artificial Sequence
  source: /note="Description of Artificial Sequence: Synthetic peptide"
NYIH

SEQ ID NO: 319 - protein, 5 aa, Artificial Sequence
  source: /note="Description of Artificial Sequence: Synthetic peptide"
NHYVH

SEQ ID NO: 320 - protein, 5 aa, Artificial Sequence
  source: /note="Description of Artificial Sequence: Synthetic peptide"
SHYMH

SEQ ID NO: 321 - protein, 5 aa, Artificial Sequence
  source: /note="Description of Artificial Sequence: Synthetic peptide"
RHLLH

SEQ ID NO: 322 - protein, 17 aa, Artificial Sequence
  source: /note="Description of Artificial Sequence: Synthetic peptide"
WMSPYNGITGYAQKFQG

SEQ ID NO: 323 - protein, 17 aa, Artificial Sequence
  source: /note="Description of Artificial Sequence: Synthetic peptide"
WMSPSSGITGYAQKFQG

SEQ ID NO: 324 - protein, 17 aa, Artificial Sequence
  source: /note="Description of Artificial Sequence: Synthetic peptide"
WMTTNSGITGYAQKFQG

SEQ ID NO: 325 - protein, 17 aa, Artificial Sequence
  source: /note="Description of Artificial Sequence: Synthetic peptide"
GIIPIFGTASYAQKFQG

SEQ ID NO: 326 - protein, 17 aa, Artificial Sequence
  source: /note="Description of Artificial Sequence: Synthetic peptide"
WMNPNSGHAGSAQKFQG

SEQ ID NO: 327 - protein, 17 aa, Artificial Sequence
  source: /note="Description of Artificial Sequence: Synthetic peptide"
WMNPNSGNTGYAQKFQG

SEQ ID NO: 328 - protein, 17 aa, Artificial Sequence
  source: /note="Description of Artificial Sequence: Synthetic peptide"
WMNPNSGNTGYSQKFQG

SEQ ID NO: 329 - protein, 17 aa, Artificial Sequence
  source: /note="Description of Artificial Sequence: Synthetic peptide"
WMNPNIGNTGYAQKFQG

SEQ ID NO: 330 - protein, 17 aa, Artificial Sequence
  source: /note="Description of Artificial Sequence: Synthetic peptide"
WMNPNGGTTGYAQNFQG

SEQ ID NO: 331 - protein, 17 aa, Artificial Sequence
  source: /note="Description of Artificial Sequence: Synthetic peptide"
WMNPNRGITDSAQKFQG

SEQ ID NO: 332 - protein, 17 aa, Artificial Sequence
  source: /note="Description of Artificial Sequence: Synthetic peptide"
WMNPNSGSAGYAQKFQG

SEQ ID NO: 333 - protein, 17 aa, Artificial Sequence
  source: /note="Description of Artificial Sequence: Synthetic peptide"
WIHPRSGATGYAPKFQG

SEQ ID NO: 334 - protein, 17 aa, Artificial Sequence
  source: /note="Description of Artificial Sequence: Synthetic peptide"
WISPRSGVTSYAQKFQG

SEQ ID NO: 335 - protein, 17 aa, Artificial Sequence
  source: /note="Description of Artificial Sequence: Synthetic peptide"
WMDPNSGNTGYAQKFQG

SEQ ID NO: 336 - protein, 17 aa, Artificial Sequence
  source: /note="Description of Artificial Sequence: Synthetic peptide"
WMNPTGGITGYAQKFQG

SEQ ID NO: 337 - protein, 17 aa, Artificial Sequence
  source: /note="Description of Artificial Sequence: Synthetic peptide"
WMNPNSGHTGNAQKFQG

SEQ ID NO: 338 - protein, 17 aa, Artificial Sequence
  source: /note="Description of Artificial Sequence: Synthetic peptide"
WVSPIHGLTGYAPRFQG

SEQ ID NO: 339 - protein, 9 aa, Artificial Sequence
  source: /note="Description of Artificial Sequence: Synthetic peptide"
DRFSGSYDY

SEQ ID NO: 340 - protein, 7 aa, Artificial Sequence
  source: /note="Description of Artificial Sequence: Synthetic peptide"
DRGWFDP

SEQ ID NO: 341 - protein, 9 aa, Artificial Sequence
  source: /note="Description of Artificial Sequence: Synthetic peptide"
EGYSSGLDY

SEQ ID NO: 342 - protein, 11 aa, Artificial Sequence
  source: /note="Description of Artificial Sequence: Synthetic peptide"
DGRFWSGYPDY

SEQ ID NO: 343 - protein, 10 aa, Artificial Sequence
  source: /note="Description of Artificial Sequence: Synthetic peptide"
ESIAVAGYDY

SEQ ID NO: 344 - protein, 10 aa, Artificial Sequence
  source: /note="Description of Artificial Sequence: Synthetic peptide"
DRWYMGSADY

SEQ ID NO: 345 - protein, 10 aa, Artificial Sequence
  source: /note="Description of Artificial Sequence: Synthetic peptide"
DDWGGDWFDP

SEQ ID NO: 346 - protein, 10 aa, Artificial Sequence
  source: /note="Description of Artificial Sequence: Synthetic peptide"
ERLSVAGFDY

SEQ ID NO: 347 - protein, 10 aa, Artificial Sequence
  source: /note="Description of Artificial Sequence: Synthetic peptide"
EPLQLGGFDY

SEQ ID NO: 348 - protein, 10 aa, Artificial Sequence
  source: /note="Description of Artificial Sequence: Synthetic peptide"
EGFGPNAFDI

SEQ ID NO: 349 - protein, 10 aa, Artificial Sequence
  source: /note="Description of Artificial Sequence: Synthetic peptide"
DSWYGDWFDP

SEQ ID NO: 350 - protein, 9 aa, Artificial Sequence
  source: /note="Description of Artificial Sequence: Synthetic peptide"
EVIEVGMDV

SEQ ID NO: 351 - protein, 9 aa, Artificial Sequence
  source: /note="Description of Artificial Sequence: Synthetic peptide"
EAWFGELST

SEQ ID NO: 352 - protein, 9 aa, Artificial Sequence
  source: /note="Description of Artificial Sequence: Synthetic peptide"
EAYVAAFDI

SEQ ID NO: 353 - protein, 9 aa, Artificial Sequence
  source: /note="Description of Artificial Sequence: Synthetic peptide"
ERGYNAFDY

SEQ ID NO: 354 - protein, 8 aa, Artificial Sequence
  source: /note="Description of Artificial Sequence: Synthetic peptide"
DSVFGLDY

SEQ ID NO: 355 - protein, 10 aa, Artificial Sequence
  source: /note="Description of Artificial Sequence: Synthetic peptide"
DLDYVRAFDI

SEQ ID NO: 356 - protein, 9 aa, Artificial Sequence
  source: /note="Description of Artificial Sequence: Synthetic peptide"
ESWGGYFDL

SEQ ID NO: 357 - protein, 9 aa, Artificial Sequence
  source: /note="Description of Artificial Sequence: Synthetic peptide"
DRTTYAFDI

SEQ ID NO: 358 - protein, 9 aa, Artificial Sequence
  source: /note="Description of Artificial Sequence: Synthetic peptide"
GNWVDAFDI

SEQ ID NO: 359 - protein, 11 aa, Artificial Sequence
  source: /note="Description of Artificial Sequence: Synthetic peptide"
VHGSGSDGMDV

SEQ ID NO: 360 - protein, 11 aa, Artificial Sequence
  source: /note="Description of Artificial Sequence: Synthetic peptide"
RASQSISSWLA

SEQ ID NO: 361 - protein, 11 aa, Artificial Sequence
  source: /note="Description of Artificial Sequence: Synthetic peptide"
RASQSVGTWLA

SEQ ID NO: 362 - protein, 11 aa, Artificial Sequence
  source: /note="Description of Artificial Sequence: Synthetic peptide"
RASQGISNYLA

SEQ ID NO: 363 - protein, 11 aa, Artificial Sequence
  source: /note="Description of Artificial Sequence: Synthetic peptide"
RASQSISTWLA

SEQ ID NO: 364 - protein, 11 aa, Artificial Sequence
  source: /note="Description of Artificial Sequence: Synthetic peptide"
QASQDISNHLN

SEQ ID NO: 365 - protein, 11 aa, Artificial Sequence
  source: /note="Description of Artificial Sequence: Synthetic peptide"
RASQGISSWLA

SEQ ID NO: 366 - protein, 11 aa, Artificial Sequence
  source: /note="Description of Artificial Sequence: Synthetic peptide"
RASESISSWLA

SEQ ID NO: 367 - protein, 11 aa, Artificial Sequence
  source: /note="Description of Artificial Sequence: Synthetic peptide"
RASQSVGSWLA

SEQ ID NO: 368 - protein, 11 aa, Artificial Sequence
  source: /note="Description of Artificial Sequence: Synthetic peptide"
RASQNISNFLN

SEQ ID NO: 369 - protein, 12 aa, Artificial Sequence
  source: /note="Description of Artificial Sequence: Synthetic peptide"
RASQSLSSSYLA

SEQ ID NO: 370 - protein, 11 aa, Artificial Sequence
  source: /note="Description of Artificial Sequence: Synthetic peptide"
RASQSISSYLN

SEQ ID NO: 371 - protein, 11 aa, Artificial Sequence
  source: /note="Description of Artificial Sequence: Synthetic peptide"
RASQSISRWLA

SEQ ID NO: 372 - protein, 11 aa, Artificial Sequence
  source: /note="Description of Artificial Sequence: Synthetic peptide"
RDSHSITTWLA

SEQ ID NO: 373 - protein, 11 aa, Artificial Sequence
  source: /note="Description of Artificial Sequence: Synthetic peptide"
RASQVIRNDLA

SEQ ID NO: 374 - protein, 11 aa, Artificial Sequence
  source: /note="Description of Artificial Sequence: Synthetic peptide"
RASQSISRYLN

SEQ ID NO: 375 - protein, 7 aa, Artificial Sequence
  source: /note="Description of Artificial Sequence: Synthetic peptide"
AASSLQS

SEQ ID NO: 376 - protein, 7 aa, Artificial Sequence
  source: /note="Description of Artificial Sequence: Synthetic peptide"
AASTLEN

SEQ ID NO: 377 - protein, 7 aa, Artificial Sequence
  source: /note="Description of Artificial Sequence: Synthetic peptide"
RASNLES

SEQ ID NO: 378 - protein, 7 aa, Artificial Sequence
  source: /note="Description of Artificial Sequence: Synthetic peptide"
AASTLQR

SEQ ID NO: 379 - protein, 7 aa, Artificial Sequence
  source: /note="Description of Artificial Sequence: Synthetic peptide"
AASTLQS

SEQ ID NO: 380 - protein, 7 aa, Artificial Sequence
  source: /note="Description of Artificial Sequence: Synthetic peptide"
GASNLQR

SEQ ID NO: 381 - protein, 7 aa, Artificial Sequence
  source: /note="Description of Artificial Sequence: Synthetic peptide"
AASNLQS

SEQ ID NO: 382 - protein, 7 aa, Artificial Sequence
  source: /note="Description of Artificial Sequence: Synthetic peptide"
GASSLQS

SEQ ID NO: 383 - protein, 7 aa, Artificial Sequence
  source: /note="Description of Artificial Sequence: Synthetic peptide"
AASHLQS

SEQ ID NO: 384 - skipped

SEQ ID NO: 385 - protein, 7 aa, Artificial Sequence
  source: /note="Description of Artificial Sequence: Synthetic peptide"
DSSSLQT

SEQ ID NO: 386 - protein, 7 aa, Artificial Sequence
  source: /note="Description of Artificial Sequence: Synthetic peptide"
AASNLES

SEQ ID NO: 387 - protein, 9 aa, Artificial Sequence
  source: /note="Description of Artificial Sequence: Synthetic peptide"
QQSYSTPYT

SEQ ID NO: 388 - protein, 9 aa, Artificial Sequence
  source: /note="Description of Artificial Sequence: Synthetic peptide"
QQSFSTPYT

SEQ ID NO: 389 - protein, 9 aa, Artificial Sequence
  source: /note="Description of Artificial Sequence: Synthetic peptide"
QQSYSTPLT

SEQ ID NO: 390 - protein, 9 aa, Artificial Sequence
  source: /note="Description of Artificial Sequence: Synthetic peptide"
QQSYSTPFT

SEQ ID NO: 391 - protein, 9 aa, Artificial Sequence
  source: /note="Description of Artificial Sequence: Synthetic peptide"
QQSYSTPIT

SEQ ID NO: 392 - protein, 9 aa, Artificial Sequence
  source: /note="Description of Artificial Sequence: Synthetic peptide"
QQYYSTPYT

SEQ ID NO: 393 - protein, 9 aa, Artificial Sequence
  source: /note="Description of Artificial Sequence: Synthetic peptide"
QQSYSLPYT

SEQ ID NO: 394 - protein, 9 aa, Artificial Sequence
  source: /note="Description of Artificial Sequence: Synthetic peptide"
HQYFTTPLT

SEQ ID NO: 395 - protein, 9 aa, Artificial Sequence
  source: /note="Description of Artificial Sequence: Synthetic peptide"
QQSYSMPYT

SEQ ID NO: 396 - protein, 9 aa, Artificial Sequence
  source: /note="Description of Artificial Sequence: Synthetic peptide"
QQSYSTPVT

SEQ ID NO: 397 - protein, 9 aa, Artificial Sequence
  source: /note="Description of Artificial Sequence: Synthetic peptide"
QHFYNTQYT

SEQ ID NO: 398 - protein, 10 aa, Artificial Sequence
  source: /note="Description of Artificial Sequence: Synthetic peptide"
QQSLQYPSHF

SEQ ID NO: 399 - protein, 30 aa, Artificial Sequence; identical to SEQ ID NO: 187
  source: /note="Description of Artificial Sequence: Synthetic polypeptide"

SEQ ID NO: 400 - protein, 30 aa, Artificial Sequence; identical to SEQ ID NO: 178
  source: /note="Description of Artificial Sequence: Synthetic polypeptide"

SEQ ID NO: 401 - protein, 30 aa, Artificial Sequence; identical to SEQ ID NO: 191
  source: /note="Description of Artificial Sequence: Synthetic polypeptide"

SEQ ID NO: 402 - protein, 30 aa, Artificial Sequence
  source: /note="Description of Artificial Sequence: Synthetic polypeptide"
QVQLVQSGAEVKEPGASVKVSCKASGYTFT

SEQ ID NO: 403 - protein, 30 aa, Artificial Sequence
  source: /note="Description of Artificial Sequence: Synthetic polypeptide"
QVQLVQSGAEVKKPGASVKVSCKASGYNFS

SEQ ID NO: 404 - skipped

SEQ ID NO: 405 - protein, 30 aa, Artificial Sequence; identical to SEQ ID NO: 189
  source: /note="Description of Artificial Sequence: Synthetic polypeptide"

SEQ ID NO: 406 - protein, 30 aa, Artificial Sequence; identical to SEQ ID NO: 190
  source: /note="Description of Artificial Sequence: Synthetic polypeptide"

SEQ ID NO: 407 - protein, 14 aa, Artificial Sequence
  source: /note="Description of Artificial Sequence: Synthetic peptide"
WVRQAPGQGLEWMG

SEQ ID NO: 408 - protein, 14 aa, Artificial Sequence
  source: /note="Description of Artificial Sequence: Synthetic peptide"
WMRQAPGQGLEWIG

SEQ ID NO: 409 - protein, 32 aa, Artificial Sequence; identical to SEQ ID NO: 196
  source: /note="Description of Artificial Sequence: Synthetic polypeptide"

SEQ ID NO: 410 - protein, 32 aa, Artificial Sequence; identical to SEQ ID NO: 199
  source: /note="Description of Artificial Sequence: Synthetic polypeptide"

SEQ ID NO: 411 - protein, 11 aa, Artificial Sequence
  source: /note="Description of Artificial Sequence: Synthetic peptide"
WGQGTLVTVSS

SEQ ID NO: 412 - protein, 11 aa, Artificial Sequence
  source: /note="Description of Artificial Sequence: Synthetic peptide"
WGQGTTVTVSS

SEQ ID NO: 413 - protein, 11 aa, Artificial Sequence
  source: /note="Description of Artificial Sequence: Synthetic peptide"
WGRGTLVTVSS

SEQ ID NO: 414 - protein, 11 aa, Artificial Sequence
  source: /note="Description of Artificial Sequence: Synthetic peptide"
WGQGTMVTVSS

SEQ ID NO: 415 - protein, 23 aa, Artificial Sequence
  source: /note="Description of Artificial Sequence: Synthetic peptide"
DIQMTQSPSSLSASVGDRVTITC

SEQ ID NO: 416 - protein, 23 aa, Artificial Sequence
  source: /note="Description of Artificial Sequence: Synthetic peptide"
EIVMTQSPATLSVSPGERATLSC

SEQ ID NO: 417 - protein, 23 aa, Artificial Sequence
  source: /note="Description of Artificial Sequence: Synthetic peptide"
DIQITHSPSSLSASVGYRLTITC

SEQ ID NO: 418 - protein, 15 aa, Artificial Sequence
  source: /note="Description of Artificial Sequence: Synthetic peptide"
WYQQKPGKAPKLLIY

SEQ ID NO: 419 - protein, 15 aa, Artificial Sequence
  source: /note="Description of Artificial Sequence: Synthetic peptide"
WYQQKPGQAPRLLIY

SEQ ID NO: 420 - protein, 15 aa, Artificial Sequence
  source: /note="Description of Artificial Sequence: Synthetic peptide"
WYHQKPWNAPKLMIY

SEQ ID NO: 421 - protein, 32 aa, Artificial Sequence; identical to SEQ ID NO: 213
  source: /note="Description of Artificial Sequence: Synthetic polypeptide"

SEQ ID NO: 422 - protein, 32 aa, Artificial Sequence; identical to SEQ ID NO: 214
  source: /note="Description of Artificial Sequence: Synthetic polypeptide"

SEQ ID NO: 423 - protein, 32 aa, Artificial Sequence; identical to SEQ ID NO: 215
  source: /note="Description of Artificial Sequence: Synthetic polypeptide"

SEQ ID NO: 424 - protein, 32 aa, Artificial Sequence; identical to SEQ ID NO: 216
  source: /note="Description of Artificial Sequence: Synthetic polypeptide"

SEQ ID NO: 425 - protein, 10 aa, Artificial Sequence
  source: /note="Description of Artificial Sequence: Synthetic peptide"
FGGGTKVEIK

SEQ ID NO: 426 - protein, 10 aa, Artificial Sequence
  source: /note="Description of Artificial Sequence: Synthetic peptide"
FGQGTKLEIK

SEQ ID NO: 427 - protein, 10 aa, Artificial Sequence
  source: /note="Description of Artificial Sequence: Synthetic peptide"
FGQGTKVEIK

SEQ ID NO: 428 - protein, 10 aa, Artificial Sequence
  source: /note="Description of Artificial Sequence: Synthetic peptide"
FGQGTRLEIK

SEQ ID NO: 429 - protein, 10 aa, Artificial Sequence
  source: /note="Description of Artificial Sequence: Synthetic peptide"
FGPGTKVDIK

SEQ ID NO: 430 - protein, 118 aa, Artificial Sequence
  source: /note="Description of Artificial Sequence: Synthetic polypeptide"
QVQLVQSGAEVKKPGASVKVSCKASGYTFSSDYMHWVRQAPGQGLEWMGWMSPYNGITGYAQKFQGRVTMTRDTSTSTVYMELSSLRSEDTAVYYCARDRFSGSYDYWGQGTLVTVSS

SEQ ID NO: 431 - protein, 116 aa, Artificial Sequence
  source: /note="Description of Artificial Sequence: Synthetic polypeptide"
QVQLVQSGAEVKKPGASVKVSCKASGYTFTGYYMHWVRQAPGQGLEWMGWMSPSSGITGYAQKFQGRVTMTRDTSTSTVYMELSSLRSEDTAVYYCARDRGWFDPWGQGTLVTVSS

SEQ ID NO: 432 - protein, 118 aa, Artificial Sequence
  source: /note="Description of Artificial Sequence: Synthetic polypeptide"
QVQLVQSGAEVKKPGASVKVSCKASGYTFSSYYMHWVRQAPGQGLEWMGWMTTNSGITGYAQKFQGRVTMTRDTSTSTVYMELSSLRSEDTAVYYCAREGYSSGLDYWGQGTLVTVSS

SEQ ID NO: 433 - protein, 120 aa, Artificial Sequence
  source: /note="Description of Artificial Sequence: Synthetic polypeptide"
QVQLVQSGAEVKKPGSSVKVSCKASGYTFTGYYIHWVRQAPGQGLEWMGGIIPIFGTASYAQKFQGRVTITADESTSTAYMELSSLRSEDTAVYYCARDGRFWSGYPDYWGQGTLVTVSS

SEQ ID NO: 434 - protein, 119 aa, Artificial Sequence
  source: /note="Description of Artificial Sequence: Synthetic polypeptide"
QVQLVQSGAEVKKPGASVKVSCKASGYTFSTHYMHWVRQAPGQGLEWMGWMNPNSGHAGSAQKFQGRVTMTRDTSTSTVYMELSSLRSEDTAVYYCARESIAVAGYDYWGQGTLVTVSS

SEQ ID NO: 435 - protein, 119 aa, Artificial Sequence
  source: /note="Description of Artificial Sequence: Synthetic polypeptide"
QVQLVQSGAEVKKPGASVKVSCKASGYTFTSHDINWVRQAPGQGLEWMGWMNPNSGNTGYAQKFQGRVTMTRDTSTSTVYMELSSLRSEDTAVYYCARDRWYMGSADYWGQGTLVTVSS

SEQ ID NO: 436 - protein, 119 aa, Artificial Sequence
  source: /note="Description of Artificial Sequence: Synthetic polypeptide"
QVQLVQSGAEVKKPGASVKVSCKASGYTFTSYYMHWVRQAPGQGLEWMGWMNPNSGNTGYAQKFQGRVTMTRDTSTSTVYMELSSLRSEDTAVYYCARDDWGGDWFDPWGQGTLVTVSS

SEQ ID NO: 437 - protein, 119 aa, Artificial Sequence
  source: /note="Description of Artificial Sequence: Synthetic polypeptide"
QVQLVQSGAEVKKPGASVKVSCKASGYTFSTHYMHWVRQAPGQGLEWMGWMNPNSGNTGYSQKFQGRVTMTRDTSTSTVYMELSSLRSEDTAVYYCARERLSVAGFDYWGQGTLVTVSS

SEQ ID NO: 438 - protein, 119 aa, Artificial Sequence
  source: /note="Description of Artificial Sequence: Synthetic polypeptide"
QVQLVQSGAEVKEPGASVKVSCKASGYTFTDHYLHWVRQAPGQGLEWMGWMNPNIGNTGYAQKFQGRVTMTRDTSTSTVYMELSSLRSEDTAVYYCAREPLQLGGFDYWGQGTLVTVSS

SEQ ID NO: 439 - protein, 119 aa, Artificial Sequence
  source: /note="Description of Artificial Sequence: Synthetic polypeptide"
QVQLVQSGAEVKKPGASVKVSCKASGYTFTGYYMHWVRQAPGQGLEWMGWMNPNGGTTGYAQNFQGRVTMTRDTSTSTVYMELSSLRSEDTAVYYCAREGFGPNAFDIWGQGTTVTVSS

SEQ ID NO: 440 - protein, 119 aa, Artificial Sequence
  source: /note="Description of Artificial Sequence: Synthetic polypeptide"
QVQLVQSGAEVKKPGASVKVSCKASGYTFTGYYMHWVRQAPGQGLEWMGWMNPNSGNTGYAQKFQGRVTMTRDTSTSTVYMELSSLRSEDTAVYYCARDSWYGDWFDPWGQGTLVTVSS

SEQ ID NO: 441 - protein, 118 aa, Artificial Sequence
  source: /note="Description of Artificial Sequence: Synthetic polypeptide"
QVQLVQSGAEVKKPGASVKVSCKASGYTFTGYYMHWMRQAPGQGLEWIGWMSPYNGITGYAQKFQGRVTMTRDTSTSTVYMELSSLRSEDTAVYYCAREVIEVGMDVWGQGTTVTVSS

SEQ ID NO: 442 - protein, 118 aa, Artificial Sequence
  source: /note="Description of Artificial Sequence: Synthetic polypeptide"
QVQLVQSGAEVKKPGASVKVSCKASGYTFTNYYMHWVRQAPGQGLEWMGWMSPSSGITGYAQKFQGRVTMTRDTSTSTVYMELSSLRSEDTAVYYCAREAWFGELSTWGQGTLVTVSS

SEQ ID NO: 443 - protein, 118 aa, Artificial Sequence
  source: /note="Description of Artificial Sequence: Synthetic polypeptide"
QVQLVQSGAEVKKPGASVKVSCKASGYNFSAYYVHWVRQAPGQGLEWMGWMNPNRGITDSAQKFQGRVTMTRDTSTSTVYMELSSLRSEDTAVYYCAREAYVAAFDIWGQGTTVTVSS

SEQ ID NO: 444 - protein, 118 aa, Artificial Sequence
  source: /note="Description of Artificial Sequence: Synthetic polypeptide"
QVQLVQSGAEVKKPGASVKVSCKASGYTFTRHYVHWVRQAPGQGLEWMGWMNPNSGSAGYAQKFQGRVTMTRDTSTSTVYMELSSLRSEDTAVYYCARERGYNAFDYWGQGTLVTVSS

SEQ ID NO: 445 - protein, 116 aa, Artificial Sequence
  source: /note="Description of Artificial Sequence: Synthetic polypeptide"
QVQLVQSGAEVKKPGASVKVSCKASGYTLPNYIHWVRQAPGQGLEWMGWIHPRSGATGYAPKFQGRVTMTRDTSTSTVYMELSSLRSEDTAVYYCARDSVFGLDYWGQGTLVTVSS

SEQ ID NO: 446 - protein, 119 aa, Artificial Sequence; identical to SEQ ID NO: 260
  source: /note="Description of Artificial Sequence: Synthetic polypeptide"

SEQ ID NO: 447 - protein, 118 aa, Artificial Sequence; identical to SEQ ID NO: 261
  source: /note="Description of Artificial Sequence: Synthetic polypeptide"

SEQ ID NO: 448 - protein, 118 aa, Artificial Sequence; identical to SEQ ID NO: 262
  source: /note="Description of Artificial Sequence: Synthetic polypeptide"

SEQ ID NO: 449 - protein, 118 aa, Artificial Sequence; identical to SEQ ID NO: 243
  source: /note="Description of Artificial Sequence: Synthetic polypeptide"

SEQ ID NO: 450 - protein, 120 aa, Artificial Sequence; identical to SEQ ID NO: 264
  source: /note="Description of Artificial Sequence: Synthetic polypeptide"

SEQ ID NO: 451 - protein, 107 aa, Artificial Sequence
  source: /note="Description of Artificial Sequence: Synthetic polypeptide"
DIQMTQSPSSLSASVGDRVTITCRASQSISSWLAWYQQKPGKAPKLLIYAASSLQSGVPSRFSGSGSGTDFTLTISSLQPEDFATYYCQQSYSTPYTFGGGTKVEIK

SEQ ID NO: 452 - protein, 107 aa, Artificial Sequence
  source: /note="Description of Artificial Sequence: Synthetic polypeptide"
DIQMTQSPSSLSASVGDRVTITCRASQSVGTWLAWYQQKPGKAPKLLIYAASTLENGVPSRFSGSGSGTDFTLTISSLQPEDFATYYCQQSFSTPYTFGGGTKVEIK

SEQ ID NO: 453 - protein, 107 aa, Artificial Sequence; identical to SEQ ID NO: 451
  source: /note="Description of Artificial Sequence: Synthetic polypeptide"

SEQ ID NO: 454 - protein, 107 aa, Artificial Sequence
  source: /note="Description of Artificial Sequence: Synthetic polypeptide"
DIQMTQSPSSLSASVGDRVTITCRASQGISNYLAWYQQKPGKAPKLLIYRASNLESGVPSRFSGSGSGTDFTLTISSLQPEDFATYYCQQSYSTPLTFGGGTKVEIK

SEQ ID NO: 455 - protein, 107 aa, Artificial Sequence
  source: /note="Description of Artificial Sequence: Synthetic polypeptide"
DIQMTQSPSSLSASVGDRVTITCRASQSISSWLAWYQQKPGKAPKLLIYAASTLQRGVPSRFSGSGSGTDFTLTISSLQPEDFATYYCQQSYSTPYTFGQGTKLEIK

SEQ ID NO: 456 - protein, 107 aa, Artificial Sequence
  source: /note="Description of Artificial Sequence: Synthetic polypeptide"
DIQMTQSPSSLSASVGDRVTITCRASQSISTWLAWYQQKPGKAPKLLIYAASTLQSGVPSRFSGSGSGTDFTLTISSLQPEDFATYYCQQSYSTPFTFGQGTKVEIK

SEQ ID NO: 457 - protein, 107 aa, Artificial Sequence
  source: /note="Description of Artificial Sequence: Synthetic polypeptide"
DIQMTQSPSSLSASVGDRVTITCQASQDISNHLNWYQQKPGKAPKLLIYGASNLQRGVPSRFSGSGSGTDFTLTISSLQPEDFATYYCQQSYSTPITFGQGTRLEIK

SEQ ID NO: 458 - protein, 107 aa, Artificial Sequence
  source: /note="Description of Artificial Sequence: Synthetic polypeptide"
DIQMTQSPSSLSASVGDRVTITCRASQGISSWLAWYQQKPGKAPKLLIYAASSLQSGVPSRFSGSGSGTDFTLTISSLQPEDFATYYCQQSYSTPYTFGQGTKVEIK

SEQ ID NO: 459 - protein, 107 aa, Artificial Sequence
  source: /note="Description of Artificial Sequence: Synthetic polypeptide"
DIQMTQSPSSLSASVGDRVTITCRASESISSWLAWYQQKPGKAPKLLIYAASSLQSGVPSRFSGSGSGTDFTLTISSLQPEDFATYYCQQSYSTPLTFGQGTKLEIK

SEQ ID NO: 460 - protein, 107 aa, Artificial Sequence
  source: /note="Description of Artificial Sequence: Synthetic polypeptide"
DIQMTQSPSSLSASVGDRVTITCRASQSISSWLAWYQQKPGKAPKLLIYAASNLQSGVPSRFSGSGSGTDFTLTISSLQPEDFATYYCQQYYSTPYTFGQGTKVEIK

SEQ ID NO: 461 - protein, 107 aa, Artificial Sequence
  source: /note="Description of Artificial Sequence: Synthetic polypeptide"
DIQMTQSPSSLSASVGDRVTITCRASQSVGSWLAWYQQKPGKAPKLLIYGASSLQSGVPSRFSGSGSGTDFTLTISSLQPEDFATYYCQQSYSTPLTFGGGTKVEIK

SEQ ID NO: 462 - protein, 107 aa, Artificial Sequence
  source: /note="Description of Artificial Sequence: Synthetic polypeptide"
DIQMTQSPSSLSASVGDRVTITCRASQSISSWLAWYQQKPGKAPKLLIYAASHLQSGVPSRFSGSGSGTDFTLTISSLQPEDFATYYCQQSYSTPYTFGQGTRLEIK

SEQ ID NO: 463 - protein, 107 aa, Artificial Sequence
  source: /note="Description of Artificial Sequence: Synthetic polypeptide"
DIQMTQSPSSLSASVGDRVTITCRASQNISNFLNWYQQKPGKAPKLLIYAASSLQSGVPSRFSGSGSGTDFTLTISSLQPEDFATYYCQQSYSLPYTFGQGTKVEIK

SEQ ID NO: 464 - protein, 107 aa, Artificial Sequence
  source: /note="Description of Artificial Sequence: Synthetic polypeptide"
DIQMTQSPSSLSASVGDRVTITCRASQGISSWLAWYQQKPGKAPKLLIYAASSLQSGVPSRFSGSGSGTDFTLTISSLQPEDFATYYCQQSYSTPLTFGGGTKVEIK

SEQ ID NO: 465 - protein, 108 aa, Artificial Sequence
  source: /note="Description of Artificial Sequence: Synthetic polypeptide"
EIVMTQSPATLSVSPGERATLSCRASQSLSSSYLAWYQQKPGQAPRLLIYGASTRATGIPARFSGSGSGTEFTLTISSLQSEDFAVYYCHQYFTTPLTFGQGTRLEIK

SEQ ID NO: 466 - protein, 107 aa, Artificial Sequence
  source: /note="Description of Artificial Sequence: Synthetic polypeptide"
DIQMTQSPSSLSASVGDRVTITCRASQSISSYLNWYQQKPGKAPKLLIYAASTLQSGVPSRFSGSGSGTDFTLTISSLQPEDFATYYCQQSYSMPYTFGQGTKLEIK

SEQ ID NO: 467 - protein, 107 aa, Artificial Sequence; identical to SEQ ID NO: 302
  source: /note="Description of Artificial Sequence: Synthetic polypeptide"

SEQ ID NO: 468 - protein, 107 aa, Artificial Sequence; identical to SEQ ID NO: 303
  source: /note="Description of Artificial Sequence: Synthetic polypeptide"

SEQ ID NO: 469 - protein, 107 aa, Artificial Sequence; identical to SEQ ID NO: 304
  source: /note="Description of Artificial Sequence: Synthetic polypeptide"

SEQ ID NO: 470 - protein, 108 aa, Artificial Sequence; identical to SEQ ID NO: 305
  source: /note="Description of Artificial Sequence: Synthetic polypeptide"

SEQ ID NO: 471 - protein, 107 aa, Artificial Sequence; identical to SEQ ID NO: 306
  source: /note="Description of Artificial Sequence: Synthetic polypeptide"

SEQ ID NO: 472 - protein, 106 aa, Artificial Sequence
  source: /note="Description of Artificial Sequence: Synthetic polypeptide"
DIQLTQSPSSLSASVGDRVTITCKASQDVGTSVAWYQQKPGKAPKLLIYWTSTRHTGVPSRFSGSGSGTDFTFTISSLQPEDIATYYCQQYSLYRSFGQGTKVEIK

SEQ ID NO: 473 - protein, 23 aa, Artificial Sequence
  source: /note="Description of Artificial Sequence: Synthetic peptide"
DIQLTQSPSSLSASVGDRVTITC

SEQ ID NO: 474 - protein, 11 aa, Artificial Sequence
  source: /note="Description of Artificial Sequence: Synthetic peptide"
KASQDVGTSVA

SEQ ID NO: 475 - protein, 15 aa, Artificial Sequence
  source: /note="Description of Artificial Sequence: Synthetic peptide"
WYQQKPGKAPKLLIY

SEQ ID NO: 476 - protein, 7 aa, Artificial Sequence
  source: /note="Description of Artificial Sequence: Synthetic peptide"
WTSTRHT

SEQ ID NO: 477 - protein, 32 aa, Artificial Sequence
  source: /note="Description of Artificial Sequence: Synthetic polypeptide"
GVPSRFSGSGSGTDFTFTISSLQPEDIATYYC

SEQ ID NO: 478 - protein, 8 aa, Artificial Sequence
  source: /note="Description of Artificial Sequence: Synthetic peptide"
QQYSLYRS

SEQ ID NO: 479 - protein, 10 aa, Artificial Sequence
  source: /note="Description of Artificial Sequence: Synthetic peptide"
FGQGTKVEIK

SEQ ID NO: 480 - protein, 119 aa, Artificial Sequence
  source: /note="Description of Artificial Sequence: Synthetic polypeptide"
EVQLVESGGGVVQPGRSLRLSCSSSGFDFTTYWMSWVRQAPGKGLEWVAEIHPDSSTINYAPSLKDRFTISRDNSKNTLFLQMDSLRPEDTGVYFCASLYFGFPWFAYWGQGTPVTVSS

SEQ ID NO: 481 - protein, 30 aa, Artificial Sequence
  source: /note="Description of Artificial Sequence: Synthetic polypeptide"
EVQLVESGGGVVQPGRSLRLSCSSSGFDFT

SEQ ID NO: 482 - protein, 5 aa, Artificial Sequence
  source: /note="Description of Artificial Sequence: Synthetic peptide"
TYWMS

SEQ ID NO: 483 - protein, 14 aa, Artificial Sequence
  source: /note="Description of Artificial Sequence: Synthetic peptide"
WVRQAPGKGLEWVA

SEQ ID NO: 484 - protein, 17 aa, Artificial Sequence
  source: /note="Description of Artificial Sequence: Synthetic peptide"
EIHPDSSTINYAPSLKD

SEQ ID NO: 485 - protein, 32 aa, Artificial Sequence
  source: /note="Description of Artificial Sequence: Synthetic polypeptide"
RFTISRDNSKNTLFLQMDSLRPEDTGVYFCAS

SEQ ID NO: 486 - protein, 10 aa, Artificial Sequence
  source: /note="Description of Artificial Sequence: Synthetic peptide"
LYFGFPWFAY

SEQ ID NO: 487 - protein, 11 aa, Artificial Sequence
  source: /note="Description of Artificial Sequence: Synthetic peptide"
WGQGTPVTVSS

SEQ ID NO: 488 - protein, 108 aa, Artificial Sequence
  source: /note="Description of Artificial Sequence: Synthetic polypeptide"
DIQMTQSPSSLSASVGDRVTITCKASAAVGTYVAWYQQKPGKAPKLLIYSASYRKRGVPSRFSGSGSGTDFTLTISSLQPEDFATYYCHQYYTYPLFTFGQGTKLEIK

SEQ ID NO: 489 - protein, 23 aa, Artificial Sequence
  source: /note="Description of Artificial Sequence: Synthetic peptide"
DIQMTQSPSSLSASVGDRVTITC

SEQ ID NO: 490 - protein, 11 aa, Artificial Sequence
  source: /note="Description of Artificial Sequence: Synthetic peptide"
KASAAVGTYVA

SEQ ID NO: 491 - protein, 15 aa, Artificial Sequence
  source: /note="Description of Artificial Sequence: Synthetic peptide"
WYQQKPGKAPKLLIY

SEQ ID NO: 492 - protein, 7 aa, Artificial Sequence
  source: /note="Description of Artificial Sequence: Synthetic peptide"
SASYRKR

SEQ ID NO: 493 - protein, 32 aa, Artificial Sequence; identical to SEQ ID NO: 213
  source: /note="Description of Artificial Sequence: Synthetic polypeptide"

SEQ ID NO: 494 - protein, 10 aa, Artificial Sequence
  source: /note="Description of Artificial Sequence: Synthetic peptide"
HQYYTYPLFT

SEQ ID NO: 495 - protein, 10 aa, Artificial Sequence
  source: /note="Description of Artificial Sequence: Synthetic peptide"
FGQGTKLEIK

SEQ ID NO: 496 - protein, 30 aa, Artificial Sequence; identical to SEQ ID NO: 178
  source: /note="Description of Artificial Sequence: Synthetic polypeptide"

SEQ ID NO: 497 - protein, 5 aa, Artificial Sequence
  source: /note="Description of Artificial Sequence: Synthetic peptide"
EFGMN

SEQ ID NO: 498 - protein, 14 aa, Artificial Sequence
  source: /note="Description of Artificial Sequence: Synthetic peptide"
WVRQAPGQGLEWMG

SEQ ID NO: 499 - protein, 17 aa, Artificial Sequence
  source: /note="Description of Artificial Sequence: Synthetic peptide"
WINTKTGEATYVEEFKG

SEQ ID NO: 500 - protein, 32 aa, Artificial Sequence
  source: /note="Description of Artificial Sequence: Synthetic polypeptide"
RVTFTTDTSTSTAYMELRSLRSDDTAVYYCAR

SEQ ID NO: 501 - protein, 12 aa, Artificial Sequence
  source: /note="Description of Artificial Sequence: Synthetic peptide"
WDFAYYVEAMDY

SEQ ID NO: 502 - protein, 11 aa, Artificial Sequence
  source: /note="Description of Artificial Sequence: Synthetic peptide"
WGQGTTVTVSS

SEQ ID NO: 503 - protein, 106 aa, Artificial Sequence
  source: /note="Description of Artificial Sequence: Synthetic polypeptide"
ENVLTQSPSSMSASVGDRVNIACSASSSVSYMHWFQQKPGKSPKLWIYSTSNLASGVPSRFSGSGSGTDYSLTISSMQPEDAATYYCQQRSSYPLTFGGGTKLEIK

SEQ ID NO: 504 - protein, 23 aa, Artificial Sequence
  source: /note="Description of Artificial Sequence: Synthetic peptide"
ENVLTQSPSSMSASVGDRVNIAC

SEQ ID NO: 505 - protein, 10 aa, Artificial Sequence
  source: /note="Description of Artificial Sequence: Synthetic peptide"
SASSSVSYMH

SEQ ID NO: 506 - protein, 15 aa, Artificial Sequence
  source: /note="Description of Artificial Sequence: Synthetic peptide"
WFQQKPGKSPKLWIY

SEQ ID NO: 507 - protein, 7 aa, Artificial Sequence
  source: /note="Description of Artificial Sequence: Synthetic peptide"
STSNLAS

SEQ ID NO: 508 - protein, 32 aa, Artificial Sequence
  source: /note="Description of Artificial Sequence: Synthetic polypeptide"
GVPSRFSGSGSGTDYSLTISSMQPEDAATYYC

SEQ ID NO: 509 - protein, 9 aa, Artificial Sequence
  source: /note="Description of Artificial Sequence: Synthetic peptide"
QQRSSYPLT

SEQ ID NO: 510 - protein, 10 aa, Artificial Sequence
  source: /note="Description of Artificial Sequence: Synthetic peptide"
FGGGTKLEIK

SEQ ID NO: 511 - protein, 120 aa, Artificial Sequence
  source: /note="Description of Artificial Sequence: Synthetic polypeptide"
QVKLEQSGAEVVKPGASVKLSCKASGFNIKDSYMHWLRQGPGQRLEWIGWIDPENGDTEYAPKFQGKATFTTDTSANTAYLGLSSLRPEDTAVYYCNEGTPTGPYYFDYWGQGTLVTVSS

SEQ ID NO: 512 - protein, 30 aa, Artificial Sequence
  source: /note="Description of Artificial Sequence: Synthetic polypeptide"
QVKLEQSGAEVVKPGASVKLSCKASGFNIK

SEQ ID NO: 513 - protein, 5 aa, Artificial Sequence
  source: /note="Description of Artificial Sequence: Synthetic peptide"
DSYMH

SEQ ID NO: 514 - protein, 14 aa, Artificial Sequence
  source: /note="Description of Artificial Sequence: Synthetic peptide"
WLRQGPGQRLEWIG

SEQ ID NO: 515 - protein, 17 aa, Artificial Sequence
  source: /note="Description of Artificial Sequence: Synthetic peptide"
WIDPENGDTEYAPKFQG

SEQ ID NO: 516 - protein, 32 aa, Artificial Sequence
  source: /note="Description of Artificial Sequence: Synthetic polypeptide"
KATFTTDTSANTAYLGLSSLRPEDTAVYYCNE

SEQ ID NO: 517 - protein, 11 aa, Artificial Sequence
  source: /note="Description of Artificial Sequence: Synthetic peptide"
GTPTGPYYFDY

SEQ ID NO: 518 - protein, 11 aa, Artificial Sequence
  source: /note="Description of Artificial Sequence: Synthetic peptide"
WGQGTLVTVSS

SEQ ID NO: 519 - protein, 106 aa, Artificial Sequence
  source: /note="Description of Artificial Sequence: Synthetic polypeptide"
ENVLTQSPSSMSVSVGDRVTIACSASSSVPYMHWLQQKPGKSPKLLIYLTSNLASGVPSRFSGSGSGTDYSLTISSVQPEDAATYYCQQRSSYPLTFGGGTKLEIK

SEQ ID NO: 520 - protein, 23 aa, Artificial Sequence
  source: /note="Description of Artificial Sequence: Synthetic peptide"
ENVLTQSPSSMSVSVGDRVTIAC

SEQ ID NO: 521 - protein, 10 aa, Artificial Sequence
  source: /note="Description of Artificial Sequence: Synthetic peptide"
SASSSVPYMH

SEQ ID NO: 522 - protein, 15 aa, Artificial Sequence
  source: /note="Description of Artificial Sequence: Synthetic peptide"
WLQQKPGKSPKLLIY

SEQ ID NO: 523 - protein, 7 aa, Artificial Sequence
  source: /note="Description of Artificial Sequence: Synthetic peptide"
LTSNLAS

SEQ ID NO: 524 - protein, 32 aa, Artificial Sequence
  source: /note="Description of Artificial Sequence: Synthetic polypeptide"
GVPSRFSGSGSGTDYSLTISSVQPEDAATYYC

SEQ ID NO: 525 - protein, 9 aa, Artificial Sequence
  source: /note="Description of Artificial Sequence: Synthetic peptide"
QQRSSYPLT

SEQ ID NO: 526 - protein, 10 aa, Artificial Sequence
  source: /note="Description of Artificial Sequence: Synthetic peptide"
FGGGTKLEIK

SEQ ID NO: 527 - protein, 120 aa, Artificial Sequence; identical to SEQ ID NO: 511
  source: /note="Description of Artificial Sequence: Synthetic polypeptide"

SEQ ID NO: 528 - protein, 30 aa, Artificial Sequence; identical to SEQ ID NO: 512
  source: /note="Description of Artificial Sequence: Synthetic polypeptide"

SEQ ID NO: 529 - protein, 5 aa, Artificial Sequence
  source: /note="Description of Artificial Sequence: Synthetic peptide"
DSYMH

SEQ ID NO: 530 - protein, 14 aa, Artificial Sequence
  source: /note="Description of Artificial Sequence: Synthetic peptide"
WLRQGPGQRLEWIG

SEQ ID NO: 531 - protein, 17 aa, Artificial Sequence
  source: /note="Description of Artificial Sequence: Synthetic peptide"
WIDPENGDTEYAPKFQG

SEQ ID NO: 532 - protein, 32 aa, Artificial Sequence; identical to SEQ ID NO: 516
  source: /note="Description of Artificial Sequence: Synthetic polypeptide"

SEQ ID NO: 533 - protein, 11 aa, Artificial Sequence
  source: /note="Description of Artificial Sequence: Synthetic peptide"
GTPTGPYYFDY

SEQ ID NO: 534 - protein, 11 aa, Artificial Sequence
  source: /note="Description of Artificial Sequence: Synthetic peptide"
WGQGTLVTVSS

SEQ ID NO: 535 - protein, 23 aa, Artificial Sequence
  source: /note="Description of Artificial Sequence: Synthetic peptide"
QTVLSQSPAILSASPGEKVTMTC

SEQ ID NO: 536 - protein, 10 aa, Artificial Sequence
  source: /note="Description of Artificial Sequence: Synthetic peptide"
RASSSVTYIH

SEQ ID NO: 537 - protein, 15 aa, Artificial Sequence
  source: /note="Description of Artificial Sequence: Synthetic peptide"
WYQQKPGSSPKSWIY

SEQ ID NO: 538 - protein, 7 aa, Artificial Sequence
  source: /note="Description of Artificial Sequence: Synthetic peptide"
ATSNLAS

SEQ ID NO: 539 - protein, 32 aa, Artificial Sequence
  source: /note="Description of Artificial Sequence: Synthetic polypeptide"
GVPARFSGSGSGTSYSLTISRVEAEDAATYYC

SEQ ID NO: 540 - protein, 9 aa, Artificial Sequence
  source: /note="Description of Artificial Sequence: Synthetic peptide"
QHWSSKPPT

SEQ ID NO: 541 - protein, 10 aa, Artificial Sequence
  source: /note="Description of Artificial Sequence: Synthetic peptide"
FGGGTKLEIK

SEQ ID NO: 542 - protein, 121 aa, Artificial Sequence
  source: /note="Description of Artificial Sequence: Synthetic polypeptide"
EVKLVESGGGLVQPGGSLRLSCATSGFTFTDYYMNWVRQPPGKALEWLGFIGNKANGYTTEYSASVKGRFTISRDKSQSILYLQMNTLRAEDSATYYCTRDRGLRFYFDYWGQGTTLTVSS

SEQ ID NO: 543 - protein, 30 aa, Artificial Sequence
  source: /note="Description of Artificial Sequence: Synthetic polypeptide"
EVKLVESGGGLVQPGGSLRLSCATSGFTFT

SEQ ID NO: 544 - protein, 5 aa, Artificial Sequence
  source: /note="Description of Artificial Sequence: Synthetic peptide"
DYYMN

SEQ ID NO: 545 - protein, 14 aa, Artificial Sequence
  source: /note="Description of Artificial Sequence: Synthetic peptide"
WVRQPPGKALEWLG

SEQ ID NO: 546 - protein, 19 aa, Artificial Sequence
  source: /note="Description of Artificial Sequence: Synthetic peptide"
FIGNKANGYTTEYSASVKG

SEQ ID NO: 547 - protein, 32 aa, Artificial Sequence
  source: /note="Description of Artificial Sequence: Synthetic polypeptide"
RFTISRDKSQSILYLQMNTLRAEDSATYYCTR

SEQ ID NO: 548 - protein, 10 aa, Artificial Sequence
  source: /note="Description of Artificial Sequence: Synthetic peptide"
DRGLRFYFDY

SEQ ID NO: 549 - protein, 11 aa, Artificial Sequence
  source: /note="Description of Artificial Sequence: Synthetic peptide"
WGQGTTLTVSS

SEQ ID NO: 550 - protein, 111 aa, Artificial Sequence
  source: /note="Description of Artificial Sequence: Synthetic polypeptide"
DIQLTQSPSSLSASVGDRVTITCRAGESVDIFGVGFLHWYQQKPGKAPKLLIYRASNLESGVPSRFSGSGSRTDFTLTISSLQPEDFATYYCQQTNEDPYTFGQGTKVEIK

SEQ ID NO: 551 - protein, 23 aa, Artificial Sequence
  source: /note="Description of Artificial Sequence: Synthetic peptide"
DIQLTQSPSSLSASVGDRVTITC

SEQ ID NO: 552 - protein, 15 aa, Artificial Sequence
  source: /note="Description of Artificial Sequence: Synthetic peptide"
RAGESVDIFGVGFLH

SEQ ID NO: 553 - protein, 15 aa, Artificial Sequence
  source: /note="Description of Artificial Sequence: Synthetic peptide"
WYQQKPGKAPKLLIY

SEQ ID NO: 554 - protein, 7 aa, Artificial Sequence
  source: /note="Description of Artificial Sequence: Synthetic peptide"
RASNLES

SEQ ID NO: 555 - protein, 32 aa, Artificial Sequence
  source: /note="Description of Artificial Sequence: Synthetic polypeptide"
GVPSRFSGSGSRTDFTLTISSLQPEDFATYYC

SEQ ID NO: 556 - protein, 9 aa, Artificial Sequence
  source: /note="Description of Artificial Sequence: Synthetic peptide"
QQTNEDPYT

SEQ ID NO: 557 - protein, 10 aa, Artificial Sequence
  source: /note="Description of Artificial Sequence: Synthetic peptide"
FGQGTKVEIK

SEQ ID NO: 558 - protein, 121 aa, Artificial Sequence
  source: /note="Description of Artificial Sequence: Synthetic polypeptide"
EVQLVESGGGLVQPGGSLRLSCAASGFNIKDTYMHWVRQAPGKGLEWVARIDPANGNSKYADSVKGRFTISADTSKNTAYLQMNSLRAEDTAVYYCAPFGYYVSDYAMAYWGQGTLVTVSS

SEQ ID NO: 559 - protein, 30 aa, Artificial Sequence
  source: /note="Description of Artificial Sequence: Synthetic polypeptide"
EVQLVESGGGLVQPGGSLRLSCAASGFNIK

SEQ ID NO: 560 - protein, 5 aa, Artificial Sequence
  source: /note="Description of Artificial Sequence: Synthetic peptide"
DTYMH

SEQ ID NO: 561 - protein, 14 aa, Artificial Sequence
  source: /note="Description of Artificial Sequence: Synthetic peptide"
WVRQAPGKGLEWVA

SEQ ID NO: 562 - protein, 17 aa, Artificial Sequence
  source: /note="Description of Artificial Sequence: Synthetic peptide"
RIDPANGNSKYADSVKG

SEQ ID NO: 563 - protein, 32 aa, Artificial Sequence
  source: /note="Description of Artificial Sequence: Synthetic polypeptide"
RFTISADTSKNTAYLQMNSLRAEDTAVYYCAP

SEQ ID NO: 564 - protein, 12 aa, Artificial Sequence
  source: /note="Description of Artificial Sequence: Synthetic peptide"
FGYYVSDYAMAY

SEQ ID NO: 565 - protein, 11 aa, Artificial Sequence
  source: /note="Description of Artificial Sequence: Synthetic peptide"
WGQGTLVTVSS

SEQ ID NO: 566 - protein, 107 aa, Artificial Sequence [sequence omitted]

SEQ ID NO: 567 - protein, 23 aa, Artificial Sequence
  source: /note="Description of Artificial Sequence: Synthetic peptide"
DIQMTQSPASLSASVGDRVTITC

SEQ ID NO: 568 - protein, 11 aa, Artificial Sequence
  source: /note="Description of Artificial Sequence: Synthetic peptide"
RASENIFSYLA

SEQ ID NO: 569 - protein, 15 aa, Artificial Sequence
  source: /note="Description of Artificial Sequence: Synthetic peptide"
WYQQKPGKSPKLLVY

SEQ ID NO: 570 - protein, 7 aa, Artificial Sequence
  source: /note="Description of Artificial Sequence: Synthetic peptide"
NTRTLAE

SEQ ID NO: 571 - protein, 32 aa, Artificial Sequence
  source: /note="Description of Artificial Sequence: Synthetic polypeptide"
GVPSRFSGSGSGTDFSLTISSLQPEDFATYYC

SEQ ID NO: 572 - protein, 9 aa, Artificial Sequence
  source: /note="Description of Artificial Sequence: Synthetic peptide"
QHHYGTPFT

SEQ ID NO: 573 - protein, 10 aa, Artificial Sequence
  source: /note="Description of Artificial Sequence: Synthetic peptide"
FGSGTKLEIK

SEQ ID NO: 574 - protein, 120 aa, Artificial Sequence [sequence omitted]

SEQ ID NO: 575 - protein, 30 aa, Artificial Sequence
  source: /note="Description of Artificial Sequence: Synthetic polypeptide"
EVQLQESGPGLVKPGGSLSLSCAASGFVFS

SEQ ID NO: 576 - protein, 5 aa, Artificial Sequence
  source: /note="Description of Artificial Sequence: Synthetic peptide"
SYDMS

SEQ ID NO: 577 - protein, 14 aa, Artificial Sequence
  source: /note="Description of Artificial Sequence: Synthetic peptide"
WVRQTPERGLEWVA

SEQ ID NO: 578 - protein, 17 aa, Artificial Sequence
  source: /note="Description of Artificial Sequence: Synthetic peptide"
YISSGGGITYAPSTVKG

SEQ ID NO: 579 - protein, 32 aa, Artificial Sequence
  source: /note="Description of Artificial Sequence: Synthetic polypeptide"
RFTVSRDNAKNTLYLQMNSLTSEDTAVYYCAA

SEQ ID NO: 580 - protein, 11 aa, Artificial Sequence
  source: /note="Description of Artificial Sequence: Synthetic peptide"
HYFGSSGPFAY

SEQ ID NO: 581 - protein, 11 aa, Artificial Sequence
  source: /note="Description of Artificial Sequence: Synthetic peptide"
WGQGTLVTVSS

SEQ ID NO: 582 - protein, 116 aa, Artificial Sequence
  source: /note="Description of Artificial Sequence: Synthetic polypeptide"
QAVLTQPASLSASPGASASLTCTLRRGINVGAYSIYWYQQKPGSPPQYLLRYKSDSDKQQGSGVSSRFSASKDASANAGILLISGLQSEDEADYYCMIWHSGASAVFGGGTKLTVL

SEQ ID NO: 583 - protein, 22 aa, Artificial Sequence
  source: /note="Description of Artificial Sequence: Synthetic peptide"
QAVLTQPASLSASPGASASLTC

SEQ ID NO: 584 - protein, 14 aa, Artificial Sequence
  source: /note="Description of Artificial Sequence: Synthetic peptide"
TLRRGINVGAYSIY

SEQ ID NO: 585 - protein, 15 aa, Artificial Sequence
  source: /note="Description of Artificial Sequence: Synthetic peptide"
WYQQKPGSPPQYLLR

SEQ ID NO: 586 - protein, 11 aa, Artificial Sequence
  source: /note="Description of Artificial Sequence: Synthetic peptide"
YKSDSDKQQGS

SEQ ID NO: 587 - protein, 34 aa, Artificial Sequence
  source: /note="Description of Artificial Sequence: Synthetic polypeptide"
GVSSRFSASKDASANAGILLISGLQSEDEADYYC

SEQ ID NO: 588 - protein, 10 aa, Artificial Sequence
  source: /note="Description of Artificial Sequence: Synthetic peptide"
MIWHSGASAV

SEQ ID NO: 589 - protein, 10 aa, Artificial Sequence
  source: /note="Description of Artificial Sequence: Synthetic peptide"
FGGGTKLTVL

SEQ ID NO: 590 - protein, 121 aa, Artificial Sequence
  source: /note="Description of Artificial Sequence: Synthetic polypeptide"
EVQLVESGGGLVQPGRSLRLSCAASGFTVSSYWMHWVRQAPGKGLEWVGFIRNKANGGTTEYAASVKGRFTISRDDSKNTLYLQMNSLRAEDTAVYYCARDRGLRFYFDYWGQGTTVTVSS

SEQ ID NO: 591 - protein, 30 aa, Artificial Sequence
  source: /note="Description of Artificial Sequence: Synthetic polypeptide"
EVQLVESGGGLVQPGRSLRLSCAASGFTVS

SEQ ID NO: 592 - protein, 5 aa, Artificial Sequence
  source: /note="Description of Artificial Sequence: Synthetic peptide"
SYWMH

SEQ ID NO: 593 - protein, 14 aa, Artificial Sequence
  source: /note="Description of Artificial Sequence: Synthetic peptide"
WVRQAPGKGLEWVG

SEQ ID NO: 594 - protein, 19 aa, Artificial Sequence
  source: /note="Description of Artificial Sequence: Synthetic peptide"
FIRNKANGGTTEYAASVKG

SEQ ID NO: 595 - protein, 19 aa, Artificial Sequence
  source: /note="Description of Artificial Sequence: Synthetic peptide"
FIRNKANSGTTEYAASVKG

SEQ ID NO: 596 - protein, 32 aa, Artificial Sequence
  source: /note="Description of Artificial Sequence: Synthetic polypeptide"
RFTISRDDSKNTLYLQMNSLRAEDTAVYYCAR

SEQ ID NO: 597 - protein, 10 aa, Artificial Sequence
  source: /note="Description of Artificial Sequence: Synthetic peptide"
DRGLRFYFDY

SEQ ID NO: 598 - protein, 11 aa, Artificial Sequence
  source: /note="Description of Artificial Sequence: Synthetic peptide"
WGQGTTVTVSS

SEQ ID NO: 599 - protein, 121 aa, Artificial Sequence
  source: /note="Description of Artificial Sequence: Synthetic polypeptide"
EVQLVESGGGLVQPGRSLRLSCAASGFTVSSYWMHWVRQAPGKGLEWVGFILNKANGGTTEYAASVKGRFTISRDDSKNTLYLQMNSLRAEDTAVYYCARDRGLRFYFDYWGQGTTVTVSS

SEQ ID NO: 600 - protein, 30 aa, Artificial Sequence; identical to SEQ ID NO: 591
  source: /note="Description of Artificial Sequence: Synthetic polypeptide"

SEQ ID NO: 601 - protein, 5 aa, Artificial Sequence
  source: /note="Description of Artificial Sequence: Synthetic peptide"
SYWMH

SEQ ID NO: 602 - protein, 14 aa, Artificial Sequence
  source: /note="Description of Artificial Sequence: Synthetic peptide"
WVRQAPGKGLEWVG

SEQ ID NO: 603 - protein, 19 aa, Artificial Sequence
  source: /note="Description of Artificial Sequence: Synthetic peptide"
FILNKANGGTTEYAASVKG

SEQ ID NO: 604 - protein, 32 aa, Artificial Sequence; identical to SEQ ID NO: 596
  source: /note="Description of Artificial Sequence: Synthetic polypeptide"

SEQ ID NO: 605 - protein, 10 aa, Artificial Sequence
  source: /note="Description of Artificial Sequence: Synthetic peptide"
DRGLRFYFDY

SEQ ID NO: 606 - protein, 11 aa, Artificial Sequence
  source: /note="Description of Artificial Sequence: Synthetic peptide"
WGQGTTVTVSS

SEQ ID NO: 607 - protein, 30 aa, Artificial Sequence
  source: /note="Description of Artificial Sequence: Synthetic polypeptide"
QVQLVQSGAEVKKPGASVKVSCKASGYTLP